European Patent Specification EP 3 626 309 B1, published March 8, 2023. Title: MicroRNAs that Suppress Human Melanoma. Applicant: THE ROCKEFELLER UNIVERSITY. The sequence listing filed with the application follows.

SEQUENCE LISTING (141 sequences)

SEQ ID NO: 1 - DNA, 1223 bp, Homo sapiens
gggatccttgagtcctactcagccccagcggaggtgaaggacgtccttccccaggagccgactggccaatcacaggcaggaagatgaaggttctgtgggctgcgttgctggtcacattcctggcaggatgccaggccaaggtggagcaagcggtggagacagagccggagcccgagctgcgccagcagaccgagtggcagagcggccagcgctgggaactggcactgggtcgcttttgggattacctgcgctgggtgcagacactgtctgagcaggtgcaggaggagctgctcagctcccaggtcacccaggaactgagggcgctgatggacgagaccatgaaggagttgaaggcctacaaatcggaactggaggaacaactgaccccggtggcggaggagacgcgggcacggctgtccaaggagctgcaggcggcgcaggcccggctgggcgcggacatggaggacgtgtgcggccgcctggtgcagtaccgcggcgaggtgcaggccatgctcggccagagcaccgaggagctgcgggtgcgcctcgcctcccacctgcgcaagctgcgtaagcggctcctccgcgatgccgatgacctgcagaagcgcctggcagtgtaccaggccggggcccgcgagggcgccgagcgcggcctcagcgccatccgcgagcgcctggggcccctggtggaacagggccgcgtgcgggccgccactgtgggctccctggccggccagccgctacaggagcgggcccaggcctggggcgagcggctgcgcgcgcggatggaggagatgggcagccggacccgcgaccgcctggacgaggtgaaggagcaggtggcggaggtgcgcgccaagctggaggagcaggcccagcagatacgcctgcaggccgaggccttccaggcccgcctcaagagctggttcgagcccctggtggaagacatgcagcgccagtgggccgggctggtggagaaggtgcaggctgccgtgggcaccagcgccgcccctgtgcccagcgacaatcactgaacgccgaagcctgcagccatgcgaccccacgccaccccgtgcctcctgcctccgcgcagcctgcagcgggagaccctgtccccgccccagccgtcctcctggggtggaccctagtttaataaagattcaccaagtttcacgcaaaaaaaaaaaaaaaaaaaaaaaaaaaaaaaaaaaaaaaaaaaa

SEQ ID NO: 2 - protein, 317 aa, Homo sapiens [sequence omitted]

SEQ ID NO: 3 - RNA, 3203 nt, Homo sapiens
agucccacccuucggcgcagggcuccggccaacacagcccuccaggccgccuacucuccagccagccggcuccacggacccacggaagggcaagggggcggccucggggcggcgggacaguugucggagggcgcccuccaggcccaagccgccuucuccggcccccgccauggcccggggcggcagucagagcuggagcuccggggaaucagacgggcagccaaaggagcagacgcccgagaagcccagacacaagauggugaaggagacccaguacuaugacauccugggcgugaagcccagcgcguccccggaggagaucaagaaggccuaucggaagcuggcgcucaaguaccacccggacaagaacccggaugagggcgagaaguuuaaacucauaucccaggcauaugaagugcuuucagauccaaagaaaagggauguuuaugaccaaggcggagagcaggcaauuaaagaaggaggcucaggcagccccagcuucucuucacccauggacaucuuugacauguucuuugguggugguggacggauggcuagagagagaagaggcaagaauguuguacaccaguuaucuguaacucuugaagaucuauauaauggagucacgaagaaauuggcccuccagaaaaauguaauuugugagaaaugugaagguguuggugggaagaagggaucgguggagaagugcccgcugugcaaggggcgggggaugcagauccacauccagcagaucgggccgggcaugguacagcagauccagaccgugugcaucgagugcaagggccagggugagcgcaucaaccccaaggaccgcugcgagagcugcagcggggccaaggugauccgugagaagaagauuaucgagguacauguugaaaaagguaugaaagaugggcaaaagauacuauuucauggagaaggagaucaggagccugagcuggagccuggugaugucauaauugugcuugaucagaaggaucauagugucuuucagagacgaggccaugacuugaucaugaaaaugaaaauucagcuuucugaagcucuuuguggcuucaagaagacgauaaaaacauuggacaaucgaauucuuguuauuacauccaaagcaggugaggugauaaagcacggggaccugagaugcgugcgcgaugaaggaaugcccaucuacaaagcaccccuggaaaaagggauucugaucauacaguuuuuaguaaucuuuccugaaaaacacuggcuuucucuggaaaagcuuccucagcuggaagcuuuacucccuccucgacagaaagugaggauuacagaugacauggaucagguggagcugaaggaguuuugucccaaugagcagaacuggcgucagcacagggaggccuacgaggaggacgaagacgggccccaggcuggagugcagugccagacggcaugacguggugcggggcagcguggccccaccggacuagcacaugaugaauguaaaguuggcacaaugaaaaugacaucgcuuuaauggccuuguguuugggauguccuguguauguguucagcauucuuaauugcugagugucuuuuuggcuuuucuuuugguuguaacuuaaguuauagcuuaauuuauauuuaaauguuuuaaguauaaaucaccucuagucugcauauggaaucuguucauuucuauuuucaggauauacuuuugagaugucagugauugcaccaauacuuugugcuucuaguggcuuugccauaauucagugucaccaauaaggcacagcccaguuagcagcuuagccccccuagcaaaccccaaggcacaaagugggcauccugacucaucucuaggucugugguuucuccccucuucccuuggcagaguuauugagggcaugaucucagggcugcuaagauaacauuucugaggauucuagaugauccucuuaaagaauaaaagcacauccguggaucggacauggcugcaugugccugcuuaacagggccaacuuaguuccuacuguucugugcccuucaguggauggaacgugagugucugaucaucucucuuggaaguuuucugaaccuuccaagcucuguggugaggacaaaccaguguuugaaucauaugcugauaacuguuugccugugacccucacaccuuguucuucaggguuuuaaugauuuucuguugacaacuuuugcaaugcuuucccaccaaagugcuuacuuguaaagaaaacuaaauccuucuguguccccggcagccucagugcagcaacagaagccaagggagaaugcugcugguuuggcccauggcacagccagcuucucugaccaguaauccggggugacuugagggucugcaaaggcauagaacuccccaguguuuuccaccucauucucccagauugagcucccuuccaaaggaucguuccucucauugcacagccauauuacaaaggguuuccugcucaagugauguuuugguaagaacuucgcugaguuccacuguggauuacaguuuguauggacuacuacuguaaauuauagcuuguuuggagggauauuagucauuauuuuauucaugacagguagacuacaauucgaacuuaggguuaccucagucuuuagccauuacugcuuauuucuuuuccccaagucacaaaaaacuuguaagcugcuggguuaaagcagaggccaccugucagaucuacccuacccuuauuugguuacauggcaccugagaguuucacucagaccagggaucuuccuuaggagggucaaagugcagaucagaccaugcagguaaggugaaccagcugcacggaccagguucccgcaaaacauugccagcuagugaggcauaauuugcucaaaguauagaaacagcccaccugugcccacuuugaccauuggugaggauagauauaaaaucacuucuuccaacgaagccuaggugaaaaucuauuuauaaauggaccacaacucuggggugucguuuuugugcugugacuuccuaauuauugcuaaagaacuacuguuuaguugguaaugguguaaaauuacauucagcuccuucuugucauauaaaaggaauuuggagggugucgcuuaaaauuuuauuccaccuguacauuugucacuuuaaaauuaaaauugagcugguaugagagauaaaaaaaaaaaaaaaaaaa

SEQ ID NO: 4 - protein, 426 aa, Homo sapiens
MARGGSQSWSSGESDGQPKEQTPEKPRHKMVKETQYYDILGVKPSASPEEIKKAYRKLALKYHPDKNPDEGEKFKLISQAYEVLSDPKKRDVYDQGGEQAIKEGGSGSPSFSSPMDIFDMFFGGGGRMARERRGKNVVHQLSVTLEDLYNGVTKKLALQKNVICEKCEGVGGKKGSVEKCPLCKGRGMQIHIQQIGPGMVQQIQTVCIECKGQGERINPKDRCESCSGAKVIREKKIIEVHVEKGMKDGQKILFHGEGDQEPELEPGDVIIVLDQKDHSVFQRRGHDLIMKMKIQLSEALCGFKKTIKTLDNRILVITSKAGEVIKHGDLRCVRDEGMPIYKAPLEKGILIIQFLVIFPEKHWLSLEKLPQLEALLPPRQKVRITDDMDQVELKEFCPNEQNWRQHREAYEEDEDGPQAGVQCQTA

SEQ ID NO: 5 - RNA, 3064 nt, Homo sapiens
gugaccgugacgcgcgagcgggcggcgggggcgcgggccaggggcgcgggccagggugccggcaggggcguccggggcgcucugaccggccucgcccgccccccccgcagacacaagauggugaaggagacccaguacuaugacauccugggcgugaagcccagcgcguccccggaggagaucaagaaggccuaucggaagcuggcgcucaaguaccacccggacaagaacccggaugagggcgagaaguuuaaacucauaucccaggcauaugaagugcuuucagauccaaagaaaagggauguuuaugaccaaggcggagagcaggcaauuaaagaaggaggcucaggcagccccagcuucucuucacccauggacaucuuugacauguucuuugguggugguggacggauggcuagagagagaagaggcaagaauguuguacaccaguuaucuguaacucuugaagaucuauauaauggagucacgaagaaauuggcccuccagaaaaauguaauuugugagaaaugugaagguguuggugggaagaagggaucgguggagaagugcccgcugugcaaggggcgggggaugcagauccacauccagcagaucgggccgggcaugguacagcagauccagaccgugugcaucgagugcaagggccagggugagcgcaucaaccccaaggaccgcugcgagagcugcagcggggccaaggugauccgugagaagaagauuaucgagguacauguugaaaaagguaugaaagaugggcaaaagauacuauuucauggagaaggagaucaggagccugagcuggagccuggugaugucauaauugugcuugaucagaaggaucauagugucuuucagagacgaggccaugacuugaucaugaaaaugaaaauucagcuuucugaagcucuuuguggcuucaagaagacgauaaaaacauuggacaaucgaauucuuguuauuacauccaaagcaggugaggugauaaagcacggggaccugagaugcgugcgcgaugaaggaaugcccaucuacaaagcaccccuggaaaaagggauucugaucauacaguuuuuaguaaucuuuccugaaaaacacuggcuuucucuggaaaagcuuccucagcuggaagcuuuacucccuccucgacagaaagugaggauuacagaugacauggaucagguggagcugaaggaguuuugucccaaugagcagaacuggcgucagcacagggaggccuacgaggaggacgaagacgggccccaggcuggagugcagugccagacggcaugacguggugcggggcagcguggccccaccggacuagcacaugaugaauguaaaguuggcacaaugaaaaugacaucgcuuuaauggccuuguguuugggauguccuguguauguguucagcauucuuaauugcugagugucuuuuuggcuuuucuuuugguuguaacuuaaguuauagcuuaauuuauauuuaaauguuuuaaguauaaaucaccucuagucugcauauggaaucuguucauuucuauuuucaggauauacuuuugagaugucagugauugcaccaauacuuugugcuucuaguggcuuugccauaauucagugucaccaauaaggcacagcccaguuagcagcuuagccccccuagcaaaccccaaggcacaaagugggcauccugacucaucucuaggucugugguuucuccccucuucccuuggcagaguuauugagggcaugaucucagggcugcuaagauaacauuucugaggauucuagaugauccucuuaaagaauaaaagcacauccguggaucggacauggcugcaugugccugcuuaacagggccaacuuaguuccuacuguucugugcccuucaguggauggaacgugagugucugaucaucucucuuggaaguuuucugaaccuuccaagcucuguggugaggacaaaccaguguuugaaucauaugcugauaacuguuugccugugacccucacaccuuguucuucaggguuuuaaugauuuucuguugacaacuuuugcaaugcuuucccaccaaagugcuuacuuguaaagaaaacuaaauccuucuguguccccggcagccucagugcagcaacagaagccaagggagaaugcugcugguuuggcccauggcacagccagcuucucugaccaguaauccggggugacuugagggucugcaaaggcauagaacuccccaguguuuuccaccucauucucccagauugagcucccuuccaaaggaucguuccucucauugcacagccauauuacaaaggguuuccugcucaagugauguuuugguaagaacuucgcugaguuccacuguggauuacaguuuguauggacuacuacuguaaauuauagcuuguuuggagggauauuagucauuauuuuauucaugacagguagacuacaauucgaacuuaggguuaccucagucuuuagccauuacugcuuauuucuuuuccccaagucacaaaaaacuuguaagcugcuggguuaaagcagaggccaccugucagaucuacccuacccuuauuugguuacauggcaccugagaguuucacucagaccagggaucuuccuuaggagggucaaagugcagaucagaccaugcagguaaggugaaccagcugcacggaccagguucccgcaaaacauugccagcuagugaggcauaauuugcucaaaguauagaaacagcccaccugugcccacuuugaccauuggugaggauagauauaaaaucacuucuuccaacgaagccuaggugaaaaucuauuuauaaauggaccacaacucuggggugucguuuuugugcugugacuuccuaauuauugcuaaagaacuacuguuuaguugguaaugguguaaaauuacauucagcuccuucuugucauauaaaaggaauuuggagggugucgcuuaaaauuuuauuccaccuguacauuugucacuuuaaaauuaaaauugagcugguaugagagauaaaaaaaaaaaaaaaaaaa

SEQ ID NO: 6 - protein, 397 aa, Homo sapiens
MVKETQYYDILGVKPSASPEEIKKAYRKLALKYHPDKNPDEGEKFKLISQAYEVLSDPKKRDVYDQGGEQAIKEGGSGSPSFSSPMDIFDMFFGGGGRMARERRGKNVVHQLSVTLEDLYNGVTKKLALQKNVICEKCEGVGGKKGSVEKCPLCKGRGMQIHIQQIGPGMVQQIQTVCIECKGQGERINPKDRCESCSGAKVIREKKIIEVHVEKGMKDGQKILFHGEGDQEPELEPGDVIIVLDQKDHSVFQRRGHDLIMKMKIQLSEALCGFKKTIKTLDNRILVITSKAGEVIKHGDLRCVRDEGMPIYKAPLEKGILIIQFLVIFPEKHWLSLEKLPQLEALLPPRQKVRITDDMDQVELKEFCPNEQNWRQHREAYEEDEDGPQAGVQCQTA

SEQ ID NO: 7 - RNA, 2891 nt, Homo sapiens
acauuucagcaagcuggcuaaagacaugugggaaagccugacccuggauucaggucaaaucucagcacucacaagauuuaaacucauaucccaggcauaugaagugcuuucagauccaaagaaaagggauguuuaugaccaaggcggagagcaggcaauuaaagaaggaggcucaggcagccccagcuucucuucacccauggacaucuuugacauguucuuugguggugguggacggauggcuagagagagaagaggcaagaauguuguacaccaguuaucuguaacucuugaagaucuauauaauggagucacgaagaaauuggcccuccagaaaaauguaauuugugagaaaugugaagguguuggugggaagaagggaucgguggagaagugcccgcugugcaaggggcgggggaugcagauccacauccagcagaucgggccgggcaugguacagcagauccagaccgugugcaucgagugcaagggccagggugagcgcaucaaccccaaggaccgcugcgagagcugcagcggggccaaggugauccgugagaagaagauuaucgagguacauguugaaaaagguaugaaagaugggcaaaagauacuauuucauggagaaggagaucaggagccugagcuggagccuggugaugucauaauugugcuugaucagaaggaucauagugucuuucagagacgaggccaugacuugaucaugaaaaugaaaauucagcuuucugaagcucuuuguggcuucaagaagacgauaaaaacauuggacaaucgaauucuuguuauuacauccaaagcaggugaggugauaaagcacggggaccugagaugcgugcgcgaugaaggaaugcccaucuacaaagcaccccuggaaaaagggauucugaucauacaguuuuuaguaaucuuuccugaaaaacacuggcuuucucuggaaaagcuuccucagcuggaagcuuuacucccuccucgacagaaagugaggauuacagaugacauggaucagguggagcugaaggaguuuugucccaaugagcagaacuggcgucagcacagggaggccuacgaggaggacgaagacgggccccaggcuggagugcagugccagacggcaugacguggugcggggcagcguggccccaccggacuagcacaugaugaauguaaaguuggcacaaugaaaaugacaucgcuuuaauggccuuguguuugggauguccuguguauguguucagcauucuuaauugcugagugucuuuuuggcuuuucuuuugguuguaacuuaaguuauagcuuaauuuauauuuaaauguuuuaaguauaaaucaccucuagucugcauauggaaucuguucauuucuauuuucaggauauacuuuugagaugucagugauugcaccaauacuuugugcuucuaguggcuuugccauaauucagugucaccaauaaggcacagcccaguuagcagcuuagccccccuagcaaaccccaaggcacaaagugggcauccugacucaucucuaggucugugguuucuccccucuucccuuggcagaguuauugagggcaugaucucagggcugcuaagauaacauuucugaggauucuagaugauccucuuaaagaauaaaagcacauccguggaucggacauggcugcaugugccugcuuaacagggccaacuuaguuccuacuguucugugcccuucaguggauggaacgugagugucugaucaucucucuuggaaguuuucugaaccuuccaagcucuguggugaggacaaaccaguguuugaaucauaugcugauaacuguuugccugugacccucacaccuuguucuucaggguuuuaaugauuuucuguugacaacuuuugcaaugcuuucccaccaaagugcuuacuuguaaagaaaacuaaauccuucuguguccccggcagccucagugcagcaacagaagccaagggagaaugcugcugguuuggcccauggcacagccagcuucucugaccaguaauccggggugacuugagggucugcaaaggcauagaacuccccaguguuuuccaccucauucucccagauugagcucccuuccaaaggaucguuccucucauugcacagccauauuacaaaggguuuccugcucaagugauguuuugguaagaacuucgcugaguuccacuguggauuacaguuuguauggacuacuacuguaaauuauagcuuguuuggagggauauuagucauuauuuuauucaugacagguagacuacaauucgaacuuaggguuaccucagucuuuagccauuacugcuuauuucuuuuccccaagucacaaaaaacuuguaagcugcuggguuaaagcagaggccaccugucagaucuacccuacccuuauuugguuacauggcaccugagaguuucacucagaccagggaucuuccuuaggagggucaaagugcagaucagaccaugcagguaaggugaaccagcugcacggaccagguucccgcaaaacauugccagcuagugaggcauaauuugcucaaaguauagaaacagcccaccugugcccacuuugaccauuggugaggauagauauaaaaucacuucuuccaacgaagccuaggugaaaaucuauuuauaaauggaccacaacucuggggugucguuuuugugcugugacuuccuaauuauugcuaaagaacuacuguuuaguugguaaugguguaaaauuacauucagcuccuucuugucauauaaaaggaauuuggagggugucgcuuaaaauuuuauuccaccuguacauuugucacuuuaaaauuaaaauugagcugguaugagagauaaaaaaaaaaaaaaaaaaa

SEQ ID NO: 8 - protein, 370 aa, Homo sapiens
MWESLTLDSGQISALTRFKLISQAYEVLSDPKKRDVYDQGGEQAIKEGGSGSPSFSSPMDIFDMFFGGGGRMARERRGKNVVHQLSVTLEDLYNGVTKKLALQKNVICEKCEGVGGKKGSVEKCPLCKGRGMQIHIQQIGPGMVQQIQTVCIECKGQGERINPKDRCESCSGAKVIREKKIIEVHVEKGMKDGQKILFHGEGDQEPELEPGDVIIVLDQKDHSVFQRRGHDLIMKMKIQLSEALCGFKKTIKTLDNRILVITSKAGEVIKHGDLRCVRDEGMPIYKAPLEKGILIIQFLVIFPEKHWLSLEKLPQLEALLPPRQKVRITDDMDQVELKEFCPNEQNWRQHREAYEEDEDGPQAGVQCQTA

SEQ ID NO: 9 - RNA, 14905 nt, Homo sapiens
cagcggugcgagcuccaggcccaugcacugaggaggcggaaacaaggggagcccccagagcuccaucaagcccccuccaaaggcuccccuacccgguccacgccccccacccccccuccccgccuccucccaauugugcauuuuugcagccggaggcggcuccgagauggggcugugagcuucgcccggggagggggaaagagcagcgaggagugaagcggggggguggggugaaggguuuggauuucggggcagggggcgcacccccgucagcaggcccuccccaaggggcucggaacucuaccucuucacccacgccccuggugcgcuuugccgaaggaaagaauaagaacagagaaggaggagggggaaaggaggaaaagggggaccccccaacuggggggggugaaggagagaaguagcaggaccagaggggaaggggcugcugcuugcaucagcccacaccaugcugaccccgccguugcuccugcugcugccccugcucucagcucuggucgcggcggcuaucgacgccccuaagacuugcagccccaagcaguuugccugcagagaucaaauaaccuguaucucaaagggcuggcggugcgacggugagagggacugcccagacggaucugacgaggccccugagauuuguccacagaguaaggcccagcgaugccagccaaacgagcauaacugccuggguacugagcuguguguucccaugucccgccucugcaaugggguccaggacugcauggacggcucagaugaggggccccacugccgagagcuccaaggcaacugcucucgccugggcugccagcaccauuguguccccacacucgaugggcccaccugcuacugcaacagcagcuuucagcuucaggcagauggcaagaccugcaaagauuuugaugagugcucaguguacggcaccugcagccagcuaugcaccaacacagacggcuccuucauauguggcuguguugaaggauaccuccugcagccggauaaccgcuccugcaaggccaagaacgagccaguagaccggcccccugugcuguugauagccaacucccagaacaucuuggccacguaccugaguggggcccaggugucuaccaucacaccuacgagcacgcggcagaccacagccauggacuucagcuaugccaacgagaccguaugcugggugcauguuggggacagugcugcucagacgcagcucaagugugcccgcaugccuggccuaaagggcuucguggaugagcacaccaucaacaucucccucagucugcaccacguggaacagauggccaucgacuggcugacaggcaacuucuacuuuguggaugacaucgaugauaggaucuuugucugcaacagaaauggggacacaugugucacauugcuagaccuggaacucuacaaccccaagggcauugcccuggacccugccauggggaagguguuuuucacugacuaugggcagaucccaaagguggaacgcugugacauggaugggcagaaccgcaccaagcucgucgacagcaagauuguguuuccucauggcaucacgcuggaccuggucagccgccuugucuacugggcagaugccuaucuggacuauauugaagugguggacuaugagggcaagggccgccagaccaucauccagggcauccugauugagcaccuguacggccugacuguguuugagaauuaucucuaugccaccaacucggacaaugccaaugcccagcagaagacgagugugauccgugugaaccgcuuuaacagcaccgaguaccagguugucacccggguggacaaggguggugcccuccacaucuaccaccagaggcgucagccccgagugaggagccaugccugugaaaacgaccaguaugggaagccggguggcugcucugacaucugccugcuggccaacagccacaaggcgcggaccugccgcugccguuccggcuucagccugggcagugacgggaagucaugcaagaagccggagcaugagcuguuccucguguauggcaagggccggccaggcaucauccggggcauggauaugggggccaaggucccggaugagcacaugauccccauugaaaaccucaugaacccccgagcccuggacuuccacgcugagaccggcuucaucuacuuugccgacaccaccagcuaccucauuggccgccagaagauugauggcacugagcgggagaccauccugaaggacggcauccacaauguggaggguguggccguggacuggaugggagacaaucuguacuggacggacgaugggcccaaaaagacaaucagcguggccaggcuggagaaagcugcucagacccgcaagacuuuaaucgagggcaaaaugacacaccccagggcuauugugguggauccacucaauggguggauguacuggacagacugggaggaggaccccaaggacagucggcgugggcggcuggagagggcguggauggauggcucacaccgagacaucuuugucaccuccaagacagugcuuuggcccaaugggcuaagccuggacaucccggcugggcgccucuacuggguggaugccuucuacgaccgcaucgagacgauacugcucaauggcacagaccggaagauuguguaugaagguccugagcugaaccacgccuuuggccugugucaccauggcaacuaccucuucuggacugaguaucggaguggcagugucuaccgcuuggaacgggguguaggaggcgcaccccccacugugacccuucugcgcagugagcggccccccaucuuugagauccgaauguaugaugcccagcagcagcaaguuggcaccaacaaaugccgggugaacaauggcggcugcagcagccugugcuuggccaccccugggagccgccagugcgccugugcugaggaccagguguuggacgcagacggcgucacuugcuuggcgaacccauccuacgugccuccaccccagugccagccaggcgaguuugccugugccaacagccgcugcauccaggagcgcuggaagugugacggagacaacgauugccuggacaacagugaugaggccccagcccucugccaucagcacaccugccccucggaccgauucaagugcgagaacaaccggugcauccccaaccgcuggcucugcgacggggacaaugacugugggaacagugaagaugaguccaaugccacuuguucagcccgcaccugcccccccaaccaguucuccugugccaguggccgcugcauccccaucuccuggacgugugaucuggaugacgacuguggggaccgcucugaugagucugcuucgugugccuaucccaccugcuucccccugacucaguuuaccugcaacaauggcagauguaucaacaucaacuggagaugcgacaaugacaaugacuguggggacaacagugacgaagccggcugcagccacuccuguucuagcacccaguucaagugcaacagcgggcguugcauccccgagcacuggaccugcgauggggacaaugacugcggagacuacagugaugagacacacgccaacugcaccaaccaggccacgaggcccccugguggcugccacacugaugaguuccagugccggcuggauggacuaugcaucccccugcgguggcgcugcgauggggacacugacugcauggacuccagcgaugagaagagcugugagggagugacccacgucugcgaucccagugucaaguuuggcugcaaggacucagcucggugcaucagcaaagcgugggugugugauggcgacaaugacugugaggauaacucggacgaggagaacugcgagucccuggccugcaggccacccucgcacccuugugccaacaacaccucagucugccugcccccugacaagcugugugauggcaacgacgacuguggcgacggcucagaugagggcgagcucugcgaccagugcucucugaauaacgguggcugcagccacaacugcucaguggcaccuggcgaaggcauuguguguuccugcccucugggcauggagcuggggcccgacaaccacaccugccagauccagagcuacugugccaagcaucucaaaugcagccaaaagugcgaccagaacaaguucagcgugaagugcuccugcuacgagggcuggguccuggaaccugacggcgagagcugccgcagccuggaccccuucaagccguucaucauuuucuccaaccgccaugaaauccggcgcaucgaucuucacaaaggagacuacagcguccuggugcccggccugcgcaacaccaucgcccuggacuuccaccucagccagagcgcccucuacuggaccgacgugguggaggacaagaucuaccgcgggaagcugcuggacaacggagcccugacuaguuucgagguggugauucaguauggccuggccacacccgagggccuggcuguagacuggauugcaggcaacaucuacuggguggagaguaaccuggaucagaucgagguggccaagcuggaugggacccuccggaccacccugcuggccggugacauugagcacccaagggcaaucgcacuggauccccgggaugggauccuguuuuggacagacugggaugccagccugccccgcauugaggcagccuccaugaguggggcugggcgccgcaccgugcaccgggagaccggcucugggggcuggcccaacgggcucaccguggacuaccuggagaagcgcauccuuuggauugacgccaggucagaugccauuuacucagcccguuacgacggcucuggccacauggaggugcuucggggacacgaguuccugucgcacccguuugcagugacgcuguacgggggggaggucuacuggacugacuggcgaacaaacacacuggcuaaggccaacaaguggaccggccacaaugucaccgugguacagaggaccaacacccagcccuuugaccugcagguguaccaccccucccgccagcccauggcucccaaucccugugaggccaaugggggccagggccccugcucccaccugugucucaucaacuacaaccggaccguguccugcgccugcccccaccucaugaagcuccacaaggacaacaccaccugcuaugaguuuaagaaguuccugcuguacgcacgucagauggagauccgagguguggaccuggaugcucccuacuacaacuacaucaucuccuucacggugcccgacaucgacaacgucacagugcuagacuacgaugcccgcgagcagcguguguacuggucugacgugcggacacaggccaucaagcgggccuucaucaacggcacaggcguggagacagucgucucugcagacuugccaaaugcccacgggcuggcuguggacugggucucccgaaaccuguucuggacaagcuaugacaccaauaagaagcagaucaauguggcccggcuggauggcuccuucaagaacgcaguggugcagggccuggagcagccccauggccuugucguccacccucugcgugggaagcucuacuggaccgauggugacaacaucagcauggccaacauggauggcagcaaucgcacccugcucuucaguggccagaagggccccgugggccuggcuauugacuucccugaaagcaaacucuacuggaucagcuccgggaaccauaccaucaaccgcugcaaccuggaugggagugggcuggaggucaucgaugccaugcggagccagcugggcaaggccaccgcccuggccaucaugggggacaagcuguggugggcugaucaggugucggaaaagaugggcacaugcagcaaggcugacggcucgggcuccgugguccuucggaacagcaccacccuggugaugcacaugaaggucuaugacgagagcauccagcuggaccauaagggcaccaaccccugcagugucaacaacggugacugcucccagcucugccugcccacgucagagacgacccgcuccugcaugugcacagccggcuauagccuccggaguggccagcaggccugcgagggcguagguuccuuucuccuguacucugugcaugagggaaucaggggaauuccccuggaucccaaugacaagucagaugcccuggucccaguguccgggaccucgcuggcugucggcaucgacuuccacgcugaaaaugacaccaucuacuggguggacaugggccugagcacgaucagccgggccaagcgggaccagacguggcgugaagacguggugaccaauggcauuggccguguggagggcauugcaguggacuggaucgcaggcaacaucuacuggacagaccagggcuuugaugucaucgaggucgcccggcucaauggcuccuuccgcuacguggugaucucccagggucuagacaagccccgggccaucaccguccacccggagaaaggguacuuguucuggacugaguggggucaguauccgcguauugagcggucucggcuagauggcacggagcguguggugcuggucaacgucagcaucagcuggcccaacggcaucucaguggacuaccaggaugggaagcuguacuggugcgaugcacggacagacaagauugaacggaucgaccuggagacaggugagaaccgcgaggugguucuguccagcaacaacauggacauguuuucagugucuguguuugaggauuucaucuacuggagugacaggacucaugccaacggcucuaucaagcgcgggagcaaagacaaugccacagacuccgugccccugcgaaccggcaucggcguccagcuuaaagacaucaaagucuucaaccgggaccggcagaaaggcaccaacgugugcgcgguggccaauggcgggugccagcagcugugccuguaccggggccgugggcagcgggccugcgccugugcccacgggaugcuggcugaagacggagcaucgugccgcgaguaugccggcuaccugcucuacucagagcgcaccauucucaagaguauccaccugucggaugagcgcaaccucaaugcgcccgugcagcccuucgaggacccugagcacaugaagaacgucaucgcccuggccuuugacuaccgggcaggcaccucuccgggcacccccaaucgcaucuucuucagcgacauccacuuugggaacauccaacagaucaacgacgauggcuccaggaggaucaccauuguggaaaacgugggcuccguggaaggccuggccuaucaccguggcugggacacucucuauuggacaagcuacacgacauccaccaucacgcgccacacaguggaccagacccgcccaggggccuucgagcgugagaccgucaucacuaugucuggagaugaccacccacgggccuucguuuuggacgagugccagaaccucauguucuggaccaacuggaaugagcagcaucccagcaucaugcgggcggcgcucucgggagccaauguccugacccuuaucgagaaggacauccguacccccaauggccuggccaucgaccaccgugccgagaagcucuacuucucugacgccacccuggacaagaucgagcggugcgaguaugacggcucccaccgcuaugugauccuaaagucagagccuguccaccccuucgggcuggccguguauggggagcacauuuucuggacugacugggugcggcgggcagugcagcgggccaacaagcacgugggcagcaacaugaagcugcugcgcguggacaucccccagcagcccaugggcaucaucgccguggccaacgacaccaacagcugugaacucucuccaugccgaaucaacaacgguggcugccaggaccugugucugcucacucaccagggccaugucaacugcucaugccgagggggccgaauccuccaggaugaccucaccugccgagcggugaauuccucuugccgagcacaagaugaguuugagugugccaauggcgagugcaucaacuucagccugaccugcgacggcgucccccacugcaaggacaaguccgaugagaagccauccuacugcaacucccgccgcugcaagaagacuuuccggcagugcagcaaugggcgcuguguguccaacaugcuguggugcaacggggccgacgacuguggggauggcucugacgagaucccuugcaacaagacagccuguggugugggcgaguuccgcugccgggacgggaccugcaucgggaacuccagccgcugcaaccaguuuguggauugugaggacgccucagaugagaugaacugcagugccaccgacugcagcagcuacuuccgccugggcgugaagggcgugcucuuccagcccugcgagcggaccucacucugcuacgcacccagcugggugugugauggcgccaaugacuguggggacuacagugaugagcgcgacugcccaggugugaaacgccccagaugcccucugaauuacuucgccugcccuagugggcgcugcauccccaugagcuggacgugugacaaagaggaugacugugaacauggcgaggacgagacccacugcaacaaguucugcucagaggcccaguuugagugccagaaccaucgcugcaucuccaagcaguggcugugugacggcagcgaugacuguggggauggcucagacgaggcugcucacugugaaggcaagacgugcggccccuccuccuucuccugcccuggcacccacgugugcguccccgagcgcuggcucugugacggugacaaagacugugcugauggugcagacgagagcaucgcagcugguugcuuguacaacagcacuugugacgaccgugaguucaugugccagaaccgccagugcauccccaagcacuucgugugugaccacgaccgugacugugcagauggcucugaugagucccccgagugugaguacccgaccugcggccccagugaguuccgcugugccaaugggcgcugucugagcucccgccagugggagugugauggcgagaaugacugccacgaccagagugacgaggcucccaagaacccacacugcaccagccaagagcacaagugcaaugccucgucacaguuccugugcagcagugggcgcuguguggcugaggcacugcucugcaacggccaggaugacuguggcgacagcucggacgagcguggcugccacaucaaugagugucucagccgcaagcucaguggcugcagccaggacugugaggaccucaagaucggcuucaagugccgcugucgcccuggcuuccggcugaaggacgacggccggacgugugcugauguggacgagugcagcaccaccuuccccugcagccagcgcugcaucaacacucauggcagcuauaagugucuguguguggagggcuaugcaccccgcggcggcgacccccacagcugcaaggcugugacugacgaggaaccguuucugaucuucgccaaccgguacuaccugcgcaagcucaaccuggacggguccaacuacacguuacuuaagcagggccugaacaacgccguugccuuggauuuugacuaccgagagcagaugaucuacuggacagaugugaccacccagggcagcaugauccgaaggaugcaccuuaacgggagcaaugugcagguccuacaccguacaggccucagcaaccccgaugggcuggcuguggacuggguggguggcaaccuguacuggugcgacaaaggccgggacaccaucgagguguccaagcucaauggggccuaucggacggugcuggucagcucuggccuccgugagcccagggcucuggugguggaugugcagaauggguaccuguacuggacagacuggggugaccauucacugaucggccgcaucggcauggauggguccagccgcagcgucaucguggacaccaagaucacauggcccaauggccugacgcuggacuaugucacugagcgcaucuacugggccgacgcccgcgaggacuacauugaauuugccagccuggauggcuccaaucgccacguugugcugagccaggacaucccgcacaucuuugcacugacccuguuugaggacuacgucuacuggaccgacugggaaacaaaguccauuaaccgagcccacaagaccacgggcaccaacaaaacgcuccucaucagcacgcugcaccggcccauggaccugcaugucuuccaugcccugcgccagccagacgugcccaaucaccccugcaaggucaacaaugguggcugcagcaaccugugccugcugucccccgggggagggcacaaaugugccugccccaccaacuucuaccugggcagcgaugggcgcaccuguguguccaacugcacggcuagccaguuuguaugcaagaacgacaagugcauccccuucugguggaagugugacaccgaggacgacugcggggaccacucagacgagcccccggacugcccugaguucaagugccggcccggacaguuccagugcuccacagguaucugcacaaacccugccuucaucugcgauggcgacaaugacugccaggacaacagugacgaggccaacugugacauccacgucugcuugcccagucaguucaaaugcaccaacaccaaccgcuguauucccggcaucuuccgcugcaaugggcaggacaacugcggagauggggaggaugagagggacugccccgaggugaccugcgcccccaaccaguuccagugcuccauuaccaaacggugcaucccccgggucugggucugcgaccgggacaaugacuguguggauggcagugaugagcccgccaacugcacccagaugaccugugguguggacgaguuccgcugcaaggauucgggccgcugcaucccagcgcguuggaagugugacggagaggaugacuguggggauggcucggaugagcccaaggaagagugugaugaacgcaccugugagccauaccaguuccgcugcaagaacaaccgcugcgugcccggccgcuggcagugcgacuacgacaacgauugcggugacaacuccgaugaagagagcugcaccccucggcccugcuccgagagugaguucuccugugccaacggccgcugcaucgcggggcgcuggaaaugcgauggagaccacgacugcgcggacggcucggacgagaaagacugcaccccccgcugugacauggaccaguuccagugcaagagcggccacugcaucccccugcgcuggcgcugugacgcagacgccgacugcauggacggcagcgacgaggaggccugcggcacuggcgugcggaccugcccccuggacgaguuccagugcaacaacaccuugugcaagccgcuggccuggaagugcgauggcgaggaugacuguggggacaacucagaugagaaccccgaggagugugcccgguucgugugcccucccaaccggcccuuccguugcaagaaugaccgcgucugucuguggaucgggcgccaaugcgauggcacggacaacuguggggaugggacugaugaagaggacugugagccccccacagcccacaccacccacugcaaagacaagaaggaguuucugugccggaaccagcgcugccucuccuccucccugcgcugcaacauguucgaugacugcggggacggcucugacgaggaggacugcagcaucgaccccaagcugaccagcugcgccaccaaugccagcaucuguggggacgaggcacgcugcgugcgcaccgagaaagcggccuacugugccugccgcucgggcuuccacaccgugcccggccagcccggaugccaagacaucaacgagugccugcgcuucggcaccugcucccagcucugcaacaacaccaagggcggccaccucugcagcugcgcucggaacuucaugaagacgcacaacaccugcaaggccgaaggcucugaguaccagguccuguacaucgcugaugacaaugagauccgcagccuguuccccggccacccccauucggcuuacgagcaggcauuccagggugacgagaguguccgcauugaugcuauggauguccaugucaaggcuggccgugucuauuggaccaacuggcacacgggcaccaucuccuaccgcagccugccaccugcugcgccuccuaccacuuccaaccgccaccggcgacagauugaccggggugucacccaccucaacauuucagggcugaagaugcccagaggcaucgccaucgacuggguggccggaaacguguacuggaccgacucgggccgagaugugauugagguggcgcagaugaagggcgagaaccgcaagacgcucaucucgggcaugauugacgagccccacgccauugugguggacccacugagggggaccauguacuggucagacuggggcaaccaccccaagauugagacggcagcgauggaugggacgcuucgggagacacuggugcaggacaacauucaguggcccacaggccuggccguggauuaucacaaugagcggcuguacugggcagacgccaagcuuucagucaucggcagcauccggcucaauggcacggaccccauuguggcugcugacagcaaacgaggccuaagucaccccuucagcaucgacgucuuugaggauuacaucuauggugucaccuacaucaauaaucgugucuucaagauccauaaguuuggccacagccccuuggucaaccugacagggggccugagccacgccucugacgugguccuuuaccaucagcacaagcagcccgaagugaccaacccaugugaccgcaagaaaugcgaguggcucugccugcugagccccagugggccugucugcaccugucccaaugggaagcggcuggacaacggcacaugcgugccugugcccucuccaacgccccccccagaugcuccccggccuggaaccuguaaccugcagugcuucaacgguggcagcuguuuccucaaugcacggaggcagcccaagugccgcugccaaccccgcuacacgggugacaagugugaacuggaccagugcugggagcacugucgcaaugggggcaccugugcugccucccccucuggcaugcccacgugccggugccccacgggcuucacgggccccaaaugcacccagcaggugugugcgggcuacugugccaacaacagcaccugcacugucaaccagggcaaccagccccagugccgaugccuacccggcuuccugggcgaccgcugccaguaccggcagugcucuggcuacugugagaacuuuggcacaugccagauggcugcugauggcucccgacaaugccgcugcacugccuacuuugagggaucgaggugugaggugaacaagugcagccgcugucucgaaggggccuguguggucaacaagcagaguggggaugucaccugcaacugcacggauggccggguggcccccagcugucugaccugcgucggccacugcagcaauggcggcuccuguaccaugaacagcaaaaugaugccugagugccagugcccaccccacaugacagggccccggugugaggagcacgucuucagccagcagcagccaggacauauagccuccauccuaaucccucugcuguugcugcugcugcugguucugguggccggagugguauucugguauaagcggcgaguccaaggggcuaagggcuuccagcaccaacggaugaccaacggggccaugaacguggagauuggaaaccccaccuacaagauguacgaaggcggagagccugaugaugugggaggccuacuggacgcugacuuugcccuggacccugacaagcccaccaacuucaccaaccccguguaugccacacucuacauggggggccauggcagucgccacucccuggccagcacggacgagaagcgagaacuccugggccggggcccugaggacgagauaggggaccccuuggcauagggcccugccccgucggacugcccccagaaagccuccugcccccugccggugaaguccuucagugagccccuccccagccagcccuucccuggccccgccggauguauaaauguaaaaaugaaggaauuacauuuuauaugugagcgagcaagccggcaagcgagcacaguauuauuucuccauccccucccugccugcuccuuggcacccccaugcugccuucagggagacaggcagggagggcuuggggcugcaccuccuacccucccaccagaacgcaccccacugggagagcugguggugcagccuuccccucccuguauaagacacuuugccaaggcucuccccucucgccccaucccugcuugcccgcucccacagcuuccugagggcuaauucugggaagggagaguucuuugcugccccugucuggaagacguggcucugggugagguaggcgggaaaggauggaguguuuuaguucuugggggaggccaccccaaaccccagccccaacuccaggggcaccuaugagauggccaugcucaaccccccucccagacaggcccucccugucuccagggcccccaccgagguucccagggcuggagacuuccucugguaaacauuccuccagccuccccuccccuggggacgccaaggaggugggccacacccaggaagggaaagcgggcagccccguuuuggggacgugaacguuuuaauaauuuuugcugaauuccuuuacaacuaaauaacacagauauuguuauaaauaaaauuguaaaaaaaaaaaaaaaaaaa

SEQ ID NO: 10 - protein, 4544 aa, Homo sapiens
MLTPPLLLLLPLLSALVAAAIDAPKTCSPKQFACRDQITCISKGWRCDGERDCPDGSDEAPEICPQSKAQRCQPNEHNCLGTELCVPMSRLCNGVQDCMDGSDEGPHCRELQGNCSRLGCQHHCVPTLDGPTCYCNSSFQLQADGKTCKDFDECSVYGTCSQLCTNTDGSFICGCVEGYLLQPDNRSCKAKNEPVDRPPVLLIANSQNILATYLSGAQVSTITPTSTRQTTAMDFSYANETVCWVHVGDSAAQTQLKCARMPGLKGFVDEHTINISLSLHHVEQMAIDWLTGNFYFVDDIDDRIFVCNRNGDTCVTLLDLELYNPKGIALDPAMGKVFFTDYGQIPKVERCDMDGQNRTKLVDSKIVFPHGITLDLVSRLVYWADAYLDYIEVVDYEGKGRQTIIQGILIEHLYGLTVFENYLYATNSDNANAQQKTSVIRVNRFNSTEYQVVTRVDKGGALHIYHQRRQPRVRSHACENDQYGKPGGCSDICLLANSHKARTCRCRSGFSLGSDGKSCKKPEHELFLVYGKGRPGIIRGMDMGAKVPDEHMIPIENLMNPRALDFHAETGFIYFADTTSYLIGRQKIDGTERETILKDGIHNVEGVAVDWMGDNLYWTDDGPKKTISVARLEKAAQTRKTLIEGKMTHPRAIVVDPLNGWMYWTDWEEDPKDSRRGRLERAWMDGSHRDIFVTSKTVLWPNGLSLDIPAGRLYWVDAFYDRIETILLNGTDRKIVYEGPELNHAFGLCHHGNYLFWTEYRSGSVYRLERGVGGAPPTVTLLRSERPPIFEIRMYDAQQQQVGTNKCRVNNGGCSSLCLATPGSRQCACAEDQVLDADGVTCLANPSYVPPPQCQPGEFACANSRCIQERWKCDGDNDCLDNSDEAPALCHQHTCPSDRFKCENNRCIPNRWLCDGDNDCGNSEDESNATCSARTCPPNQFSCASGRCIPISWTCDLDDDCGDRSDESASCAYPTCFPLTQFTCNNGRCININWRCDNDNDCGDNSDEAGCSHSCSSTQFKCNSGRCIPEHWTCDGDNDCGDYSDETHANCTNQATRPPGGCHTDEFQCRLDGLCIPLRWRCDGDTDCMDSSDEKSCEGVTHVCDPSVKFGCKDSARCISKAWVCDGDNDCEDNSDEENCESLACRPPSHPCANNTSVCLPPDKLCDGNDDCGDGSDEGELCDQCSLNNGGCSHNCSVAPGEGIVCSCPLGMELGPDNHTCQIQSYCAKHLKCSQKCDQNKFSVKCSCYEGWVLEPDGESCRSLDPFKPFIIFSNRHEIRRIDLHKGDYSVLVPGLRNTIALDFHLSQSALYWTDVVEDKIYRGKLLDNGALTSFEVVIQYGLATPEGLAVDWIAGNIYWVESNLDQIEVAKLDGTLRTTLLAGDIEHPRAIALDPRDGILFWTDWDASLPRIEAASMSGAGRRTVHRETGSGGWPNGLTVDYLEKRILWIDARSDAIYSARYDGSGHMEVLRGHEFLSHPFAVTLYGGEVYWTDWRTNTLAKANKWTGHNVTVVQRTNTQPFDLQVYHPSRQPMAPNPCEANGGQGPCSHLCLINYNRTVSCACPHLMKLHKDNTTCYEFKKFLLYARQMEIRGVDLDAPYYNYIISFTVPDIDNVTVLDYDAREQRVYWSDVRTQAIKRAFINGTGVETVVSADLPNAHGLAVDWVSRNLFWTSYDTNKKQINVARLDGSFKNAVVQGLEQPHGLVVHPLRGKLYWTDGDNISMANMDGSNRTLLFSGQKGPVGLAIDFPESKLYWISSGNHTINRCNLDGSGLEVIDAMRSQLGKATALAIMGDKLWWADQVSEKMGTCSKADGSGSVVLRNSTTLVMHMKVYDESIQLDHKGTNPCSVNNGDCSQLCLPTSETTRSCMCTAGYSLRSGQQACEGVGSFLLYSVHEGIRGIPLDPNDKSDALVPVSGTSLAVGIDFHAENDTIYWVDMGLSTISRAKRDQTWREDVVTNGIGRVEGIAVDWIAGNIYWTDQGFDVIEVARLNGSFRYVVISQGLDKPRAITVHPEKGYLFWTEWGQYPRIERSRLDGTERVVLVNVSISWPNGISVDYQDGKLYWCDARTDKIERIDLETGENREVVLSSNNMDMFSVSVFEDFIYWSDRTHANGSIKRGSKDNATDSVPLRTGIGVQLKDIKVFNRDRQKGTNVCAVANGGCQQLCLYRGRGQRACACAHGMLAEDGASCREYAGYLLYSERTILKSIHLSDERNLNAPVQPFEDPEHMKNVIALAFDYRAGTSPGTPNRIFFSDIHFGNIQQINDDGSRRITIVENVGSVEGLAYHRGWDTLYWTSYTTSTITRHTVDQTRPGAFERETVITMSGDDHPRAFVLDECQNLMFWTNWNEQHPSIMRAALSGANVLTLIEKDIRTPNGLAIDHRAEKLYFSDATLDKIERCEYDGSHRYVILKSEPVHPFGLAVYGEHIFWTDWVRRAVQRANKHVGSNMKLLRVDIPQQPMGIIAVANDTNSCELSPCRINNGGCQDLCLLTHQGHVNCSCRGGRILQDDLTCRAVNSSCRAQDEFECANGECINFSLTCDGVPHCKDKSDEKPSYCNSRRCKKTFRQCSNGRCVSNMLWCNGADDCGDGSDEIPCNKTACGVGEFRCRDGTCIGNSSRCNQFVDCEDASDEMNCSATDCSSYFRLGVKGVLFQPCERTSLCYAPSWVCDGANDCGDYSDERDCPGVKRPRCPLNYFACPSGRCIPMSWTCDKEDDCEHGEDETHCNKFCSEAQFECQNHRCISKQWLCDGSDDCGDGSDEAAHCEGKTCGPSSFSCPGTHVCVPERWLCDGDKDCADGADESIAAGCLYNSTCDDREFMCQNRQCIPKHFVCDHDRDCADGSDESPECEYPTCGPSEFRCANGRCLSSRQWECDGENDCHDQSDEAPKNPHCTSQEHKCNASSQFLCSSGRCVAEALLCNGQDDCGDSSDERGCHINECLSRKLSGCSQDCEDLKIGFKCRCRPGFRLKDDGRTCADVDECSTTFPCSQRCINTHGSYKCLCVEGYAPRGGDPHSCKAVTDEEPFLIFANRYYLRKLNLDGSNYTLLKQGLNNAVALDFDYREQMIYWTDVTTQGSMIRRMHLNGSNVQVLHRTGLSNPDGLAVDWVGGNLYWCDKGRDTIEVSKLNGAYRTVLVSSGLREPRALVVDVQNGYLYWTDWGDHSLIGRIGMDGSSRSVIVDTKITWPNGLTLDYVTERIYWADAREDYIEFASLDGSNRHVVLSQDIPHIFALTLFEDYVYWTDWETKSINRAHKTTGTNKTLLISTLHRPMDLHVFHALRQPDVPNHPCKVNNGGCSNLCLLSPGGGHKCACPTNFYLGSDGRTCVSNCTASQFVCKNDKCIPFWWKCDTEDDCGDHSDEPPDCPEFKCRPGQFQCSTGICTNPAFICDGDNDCQDNSDEANCDIHVCLPSQFKCTNTNRCIPGIFRCNGQDNCGDGEDERDCPEVTCAPNQFQCSITKRCIPRVWVCDRDNDCVDGSDEPANCTQMTCGVDEFRCKDSGRCIPARWKCDGEDDCGDGSDEPKEECDERTCEPYQFRCKNNRCVPGRWQCDYDNDCGDNSDEESCTPRPCSESEFSCANGRCIAGRWKCDGDHDCADGSDEKDCTPRCDMDQFQCKSGHCIPLRWRCDADADCMDGSDEEACGTGVRTCPLDEFQCNNTLCKPLAWKCDGEDDCGDNSDENPEECARFVCPPNRPFRCKNDRVCLWIGRQCDGTDNCGDGTDEEDCEPPTAHTTHCKDKKEFLCRNQRCLSSSLRCNMFDDCGDGSDEEDCSIDPKLTSCATNASICGDEARCVRTEKAAYCACRSGFHTVPGQPGCQDINECLRFGTCSQLCNNTKGGHLCSCARNFMKTHNTCKAEGSEYQVLYIADDNEIRSLFPGHPHSAYEQAFQGDESVRIDAMDVHVKAGRVYWTNWHTGTISYRSLPPAAPPTTSNRHRRQIDRGVTHLNISGLKMPRGIAIDWVAGNVYWTDSGRDVIEVAQMKGENRKTLISGMIDEPHAIVVDPLRGTMYWSDWGNHPKIETAAMDGTLRETLVQDNIQWPTGLAVDYHNERLYWADAKLSVIGSIRLNGTDPIVAADSKRGLSHPFSIDVFEDYIYGVTYINNRVFKIHKFGHSPLVNLTGGLSHASDVVLYHQHKQPEVTNPCDRKKCEWLCLLSPSGPVCTCPNGKRLDNGTCVPVPSPTPPPDAPRPGTCNLQCFNGGSCFLNARRQPKCRCQPRYTGDKCELDQCWEHCRNGGTCAASPSGMPTCRCPTGFTGPKCTQQVCAGYCANNSTCTVNQGNQPQCRCLPGFLGDRCQYRQCSGYCENFGTCQMAADGSRQCRCTAYFEGSRCEVNKCSRCLEGACVVNKQSGDVTCNCTDGRVAPSCLTCVGHCSNGGSCTMNSKMMPECQCPPHMTGPRCEEHVFSQQQPGHIASILIPLLLLLLLVLVAGVVFWYKRRVQGAKGFQHQRMTNGAMNVEIGNPTYKMYEGGEPDDVGGLLDADFALDPDKPTNFTNPVYATLYMGGHGSRHSLASTDEKRELLGRGPEDEIGDPLA

SEQ ID NO: 11 - RNA, 7783 nt, Homo sapiens
gcuggcggcggccgcccagggccggggccgcgcgcccagccugagcccgccccgccgccgagcgucaccgaaccugcuugaaaugcagccgaggagccggggcgggcggcagcggcggcggcggcggcggcgggggcagcggcaaccccggcgccgcggcaaggacucggagggcugagacgcggcggcggcggcgcggggagcgcggggcgcggcggccggagccccgggcccgccaugggccuccccgagccgggcccucuccggcuucuggcgcugcugcugcugcugcugcugcugcugcugcugcagcuccagcaucuugcggcggcagcggcugauccgcugcucggcggccaagggccggccaaggauugcgaaaaggaccaauuccagugccggaacgagcgcugcauccccucuguguggagaugcgacgaggacgaugacugcuuagaccacagcgacgaggacgacugccccaagaagaccugugcagacagugacuucaccugugacaacggccacugcauccacgaacgguggaagugugacggcgaggaggaguguccugauggcuccgaugaguccgaggccacuugcaccaagcagguguguccugcagagaagcugagcuguggacccaccagccacaaguguguaccugccucguggcgcugcgacggggagaaggacugcgaggguggagcggaugaggccggcugugcuaccuugugcgccccgcacgaguuccagugcggcaaccgcucgugccuggccgccguguucgugugcgacggcgacgacgacuguggugacggcagcgaugagcgcggcugugcagacccggccugcgggccccgcgaguuccgcugcggcggcgauggcggcggcgccugcaucccggagcgcugggucugcgaccgccaguuugacugcgaggaccgcucggacgaggcagccgagcucugcggccguccgggccccggggccacguccgcgcccgccgccugcgccaccgccucccaguucgccugccgcagcggcgagugcgugcaccugggcuggcgcugcgacggcgaccgcgacugcaaagacaaaucggacgaggccgacugcccacugggcaccugccguggggacgaguuccaguguggggaugggacauguguccuugcaaucaagcacugcaaccaggagcaggacuguccagaugggagugaugaagcuggcugccuacaggggcugaacgagugucugcacaacaauggcggcugcucacacaucugcacugaccucaagauuggcuuugaaugcacgugcccagcaggcuuccagcuccuggaccagaagaccuguggcgacauugaugagugcaaggacccagaugccugcagccagaucugugucaauuacaagggcuauuuuaagugugagugcuacccuggcuacgagauggaccuacugaccaagaacugcaaggcugcugcuggcaagagcccaucccuaaucuucaccaaccggcacgaggugcggaggaucgaccuggugaagcggaacuauucacgccucauccccaugcucaagaaugucguggcacuagauguggaaguugccaccaaucgcaucuacuggugugaccucuccuaccguaagaucuauagcgccuacauggacaaggccagugacccgaaagagcaggagguccucauugacgagcaguugcacucuccagagggccuggcaguggacuggguccacaagcacaucuacuggacugacucgggcaauaagaccaucucaguggccacaguugaugguggccgccgacgcacucucuucagccguaaccucagugaaccccgggccaucgcuguugacccccugcgaggguucauguauuggucugacuggggggaccaggccaagauugagaaaucugggcucaacgguguggaccggcaaacacuggugucagacaauauugaauggcccaacggaaucacccuggaucugcugagccagcgcuuguacuggguagacuccaagcuacaccaacuguccagcauugacuucaguggaggcaacagaaagacgcugaucuccuccacugacuuccugagccacccuuuugggauagcuguguuugaggacaagguguucuggacagaccuggagaacgaggccauuuucagugcaaaucggcucaauggccuggaaaucuccauccuggcugagaaccucaacaacccacaugacauugucaucuuccaugagcugaagcagccaagagcuccagaugccugugagcugaguguccagccuaauggaggcugugaauaccugugccuuccugcuccucagaucuccagccacucucccaaguacacaugugccuguccugacacaauguggcuggguccagacaugaagaggugcuaccgagcaccucaaucuaccucaacuacgacguuagcuucuaccaugacgaggacaguaccugccaccacaagagcccccgggaccaccguccacagauccaccuaccagaaccacagcacagagacaccaagccugacagcugcagucccaagcucaguuaguguccccagggcucccagcaucagcccgucuacccuaagcccugcaaccagcaaccacucccagcacuaugcaaaugaagacaguaagaugggcucaacagucacugccgcuguuaucgggaucaucgugcccauaguggugauagcccuccugugcaugaguggauaccugaucuggagaaacuggaagcggaagaacaccaaaagcaugaauuuugacaacccagucuacaggaaaacaacagaagaagaagacgaagaugagcuccauauagggagaacugcucagauuggccaugucuauccugcagcaaucagcagcuuugaucgcccacugugggcagagcccugucuuggggagaccagagaaccggaagacccagccccugcccucaaggagcuuuuugucuugccgggggaaccaaggucacagcugcaccaacucccgaagaacccucuuuccgagcugccugucgucaaauccaagcgaguggcauuaagccuugaagaugauggacuacccugaggaugggaucacccccuucgugccucauggaauucagucccaugcacuacacucuggaugguguaugacuggaugaauggguuucuauauaugggucugugugaguguaugugugugugugauuuuuuuuuuaaauuuauguugcggaaagguaaccacaaaguuaugaugaacugcaaacauccaaaggaugugagaguuuuucuauguauaauguuuuauacacuuuuuaacugguugcacuacccaugaggaauucguggaauggcuacugcugacuaacaugaugcacauaaccaaaugggggccaauggcacaguaccuuacucaucauuuaaaaacuauauuuacagaagauguuugguugcugggggggcuuuuuuagguuuuggggcauuuguuuuuuguaaauaagaugauuaugcuuuguggcuauccaucaacauaaguaaaaaaaaaaaaaaaacacuucaacucccucccccauuuagauuauuuauuaacauauuuuaaaaaucagaugaguucuauaaauaauuuagagaagugagaguauuuauuuuuggcauguuuggcccaccacacagacucuguguguguauguguguguuuauauguguaugugugugacagaaaaaucuguagagaagaggcacaucuauggcuacuguucaaauacauaaagauaaauuuauuuucacacaguccacaagggguauaucuuguaguuuucagaaaagccuuuggaaaucuggaucagaaaauagauaccaugguuugugcaauuauguaguaaaaaaggcaaaucuuuucaccucuggcuauuccugagaccccaggaagucaggaaaagccuuucagcucacccauggcugcugugacuccuaccagggcuuucuuggcuuuggcgaaggucaguguacagacauuccaugguaccagagugcucagaaacucaagauaggauaugccucacccucagcuacuccuuguuuuaaaguucagcucuuugaguaacuucuucaauuucuuucaggacacuuggguugaauucaguaaguuuccucugaagcacccugaagggugccauccuuacagagcuaaguggagacguuuccagaucagcccaaguuuacuauagagacuggcccaggcacugaaugucuaggacaugcuguggaugaagauaaagaugguggaauagguuuuaucacaucucuuauuucucuuuuccccuuacucucuaccauuuccuuuauguggggaaacauuuuaagguaauaaauagguuacuuaccaucauauguucauauagaugaaacuaauuuuuggcuuaagucagaacaacuggccaaaauugaagucauauuugaggggggaaauggcauacgcaauauuauauuauauuggauauuuauguucacacaggaauuugguuuacugcuuuguaaauaaaaggaaaaacuccggguauauguauagauguucuucauuauagacaucuucuuugcuuuucuuggccuugggggaggaagggagaagugcucuuuucuacuuguggggucucccauuggaaacauaauccuauagucccagaaggauucaguccccaguggcuuucccauccaaagagaaagaguuugaguuucuuaacucugcuguucugccacuuacucccacuagacaaccagggacaaggugcaacauggaaguguuugacuuaaguaggagcagaggagcugcaucuaaucucaucauaccuggaacuugacacacuuaagcaaaugccuucccaucccuaccugccagaugcccccaacucaaugaaguuggaugucucaccagcuugauacccuuugaauuuucagucagacauucuggaguucuagcauccuguaccuaggaccuuccucugugucacucuuggccuccuaaacucuaagaaaauaacuauauucuggagcuugggcaguguguuuugcauaauccagcaaucuccucaugacaugcauguguugauaguccugaaacauucauugagaggguaaaugcaguugaccuagaaugaccaauaccaaacagaauuuuaagaacagguggccaacuccuauggagcuuacucacauauuacuauucuuuuaagaacggaaaguaaaauuauuuuugacugaagaaaaaugaugacagugaaaaacauggaaauguacucaaaacaagugacuuuuucuguaaccuuccaaagaaacugaauuuuccaaggaauuaaaugauaacaguggcuaaggcauaguuucuaaacuuucaguaagauccuggcauucacagaaaaaaaugaugaauggggucuggacauacagccugagaucucaaaaugacaaugaaauucacaacuuuuucucagagacauucauguuuccugcauaugcuacaacugcaguuugaaagaggcagcaaugggagcaacccuuuacaagaaacaaauugugauauauucauguguuggacggcaguaaauaagaugaaaccugaggagucagauccaccuucccccauucauagaggcuuuucagccucauuuugagguacaguuacauaucuuuugccuuuugcccccgugcauagcuaucuacagccaaucacagaucacagagucacuggacuauagagcuggaaggaagcucagagacaaugccaagggggcagaaaauuuaucagaagccagucccagugcguuuccuccauuuccuucugcaggaagacuauuuugggcugccugaacauuguaucaaaccugcuaccuauacuauggucuaccuuuccuccaguggaauuacaaaggcacuaacugaaaugccuucuagaaacagagaaaacgaaacuguacuuauuuacucuugauacacagauuauuuauaaaacagauugaaguaaccuguuaacuggcaaaaagagaaugagaucggauuuaaauguauggcaguaaguccuauugaucccuccaguuaucucaguaugacugcaguauauucauucacuaaaaccacucacuagauaccaacuacacaccuggcacugcagauguaaaggucagucacacauguucugacuuuacagaguucacaguagcaguggaggaugauauauguggaaacaaaaaaggcauugauucuauucagagcacuguuagggcucaaaggagagaggggucuuuccaccuaagaaaugaggaauagggucaucauagaagugaccuuaagucuuaaaaauuaagaaggggauuccaagcugcuucagacagagacacaucgagcuaaaacacagagguaugaaagagcacagggacuuuaggaauugcacaguucauucuaacaggaacaaaaggcucaaggggggcaagaaaugaggcuguauggaaagagauucaauguaagcacuuuauaaaauagauuaauuucugauucaaugaagcauuucuugaucauuguguacaaggcacuacaugcaucauggaaaauucauuaggaugcauugccagcacuuugcagaacugauauuauucagccucaagcuuuccaguggccaaagggaaaugcugacugcuuuucauauauuugagucaaagauuuuuuauauggucaaugaagacuaauauaagggcagugggauuuucacagaugcaugccauguugucgagagccucuuagauuuucucaacugugagaaagaaaaacgaaaauguugaagacguugagucuggagaggggauacuaaucacuguccaguugggcacuggugggaauggggaaauggcacaggaaugcaagccucuccacccuaccccccgaacuccagccauacacucaucguuucacaaaauauaaaugaguuagcauuaaauguuucagaguaaauaauuccuuuucccgaaaugcaugaagauagaguaacagacuucucacacuguauuuuuaggguauggagaauuuagaagguuaaagaauuacugcuucaauuuuucaguuaaaaaaaaaucaggaagcucuguucauucaggcuaugcaccaugugcacagucaagaauuagcagaaacccucugcauuuacaaacacuuugugcuauaaaaaaguaauuuuuaaaaagccacguguguguguguguauauauauauauauauauauauuuaaagccaagguuuugauacuuuuuuacaaaaacuacaagagaaaacaaauauaccuguccaaaccauauacuuuuaaaagagcauuuuuuuuuccauacaagcuguuguuaauuuggggguaaagugcugauuugcaaacuucaucaaauuguucccaaguggauucuccuuguuugucucccccuaccaaccccaaaguuaccauauuugauguaagaaucaggcauguuagaauguugugucacacuaacugauucugcucuuuuugucuugucauucaaguuccguuagcuucuguacgcggugcccuuugcagucuggugucucuuccagaggcgagggggcugaggauggggugcugcaucucacuagcuauacuggcaucaucuugguaaacugaaaaccaaauguggacauuuguaaaaucagugcacuguuucuagagagagauuaaauucauuuaaaaaaaa

SEQ ID NO: 12 - protein, 963 aa, Homo sapiens
MGLPEPGPLRLLALLLLLLLLLLLQLQHLAAAAADPLLGGQGPAKDCEKDQFQCRNERCIPSVWRCDEDDDCLDHSDEDDCPKKTCADSDFTCDNGHCIHERWKCDGEEECPDGSDESEATCTKQVCPAEKLSCGPTSHKCVPASWRCDGEKDCEGGADEAGCATLCAPHEFQCGNRSCLAAVFVCDGDDDCGDGSDERGCADPACGPREFRCGGDGGGACIPERWVCDRQFDCEDRSDEAAELCGRPGPGATSAPAACATASQFACRSGECVHLGWRCDGDRDCKDKSDEADCPLGTCRGDEFQCGDGTCVLAIKHCNQEQDCPDGSDEAGCLQGLNECLHNNGGCSHICTDLKIGFECTCPAGFQLLDQKTCGDIDECKDPDACSQICVNYKGYFKCECYPGYEMDLLTKNCKAAAGKSPSLIFTNRHEVRRIDLVKRNYSRLIPMLKNVVALDVEVATNRIYWCDLSYRKIYSAYMDKASDPKEQEVLIDEQLHSPEGLAVDWVHKHIYWTDSGNKTISVATVDGGRRRTLFSRNLSEPRAIAVDPLRGFMYWSDWGDQAKIEKSGLNGVDRQTLVSDNIEWPNGITLDLLSQRLYWVDSKLHQLSSIDFSGGNRKTLISSTDFLSHPFGIAVFEDKVFWTDLENEAIFSANRLNGLEISILAENLNNPHDIVIFHELKQPRAPDACELSVQPNGGCEYLCLPAPQISSHSPKYTCACPDTMWLGPDMKRCYRAPQSTSTTTLASTMTRTVPATTRAPGTTVHRSTYQNHSTETPSLTAAVPSSVSVPRAPSISPSTLSPATSNHSQHYANEDSKMGSTVTAAVIGIIVPIVVIALLCMSGYLIWRNWKRKNTKSMNFDNPVYRKTTEEEDEDELHIGRTAQIGHVYPAAISSFDRPLWAEPCLGETREPEDPAPALKELFVLPGEPRSQLHQLPKNPLSELPVVKSKRVALSLEDDGLP

SEQ ID NO: 13 - RNA, 7273 nt, Homo sapiens
gcuggcggcggccgcccagggccggggccgcgcgcccagccugagcccgccccgccgccgagcgucaccgaaccugcuugaaaugcagccgaggagccggggcgggcggcagcggcggcggcggcggcggcgggggcagcggcaaccccggcgccgcggcaaggacucggagggcugagacgcggcggcggcggcgcggggagcgcggggcgcggcggccggagccccgggcccgccaugggccuccccgagccgggcccucuccggcuucuggcgcugcugcugcugcugcugcugcugcugcugcugcagcuccagcaucuugcggcggcagcggcugauccgcugcucggcggccaagggccggccaaggauugcgaaaaggaccaauuccagugccggaacgagcgcugcauccccucuguguggagaugcgacgaggacgaugacugcuuagaccacagcgacgaggacgacugccccaagaagaccugugcagacagugacuucaccugugacaacggccacugcauccacgaacgguggaagugugacggcgaggaggaguguccugauggcuccgaugaguccgaggccacuugcaccaagcagguguguccugcagagaagcugagcuguggacccaccagccacaaguguguaccugccucguggcgcugcgacggggagaaggacugcgaggguggagcggaugaggccggcugugcuaccuggcugaacgagugucugcacaacaauggcggcugcucacacaucugcacugaccucaagauuggcuuugaaugcacgugcccagcaggcuuccagcuccuggaccagaagaccuguggcgacauugaugagugcaaggacccagaugccugcagccagaucugugucaauuacaagggcuauuuuaagugugagugcuacccuggcuacgagauggaccuacugaccaagaacugcaaggcugcugcuggcaagagcccaucccuaaucuucaccaaccggcacgaggugcggaggaucgaccuggugaagcggaacuauucacgccucauccccaugcucaagaaugucguggcacuagauguggaaguugccaccaaucgcaucuacuggugugaccucuccuaccguaagaucuauagcgccuacauggacaaggccagugacccgaaagagcaggagguccucauugacgagcaguugcacucuccagagggccuggcaguggacuggguccacaagcacaucuacuggacugacucgggcaauaagaccaucucaguggccacaguugaugguggccgccgacgcacucucuucagccguaaccucagugaaccccgggccaucgcuguugacccccugcgaggguucauguauuggucugacuggggggaccaggccaagauugagaaaucugggcucaacgguguggaccggcaaacacuggugucagacaauauugaauggcccaacggaaucacccuggaucugcugagccagcgcuuguacuggguagacuccaagcuacaccaacuguccagcauugacuucaguggaggcaacagaaagacgcugaucuccuccacugacuuccugagccacccuuuugggauagcuguguuugaggacaagguguucuggacagaccuggagaacgaggccauuuucagugcaaaucggcucaauggccuggaaaucuccauccuggcugagaaccucaacaacccacaugacauugucaucuuccaugagcugaagcagccaagagcuccagaugccugugagcugaguguccagccuaauggaggcugugaauaccugugccuuccugcuccucagaucuccagccacucucccaaguacacaugugccuguccugacacaauguggcuggguccagacaugaagaggugcuaccgagcaccucaaucuaccucaacuacgacguuagcuucuaccaugacgaggacaguaccugccaccacaagagcccccgggaccaccguccacagauccaccuaccagaaccacagcacagagacaccaagccugacagcugcagucccaagcucaguuaguguccccagggcucccagcaucagcccgucuacccuaagcccugcaaccagcaaccacucccagcacuaugcaaaugaagacaguaagaugggcucaacagucacugccgcuguuaucgggaucaucgugcccauaguggugauagcccuccugugcaugaguggauaccugaucuggagaaacuggaagcggaagaacaccaaaagcaugaauuuugacaacccagucuacaggaaaacaacagaagaagaagacgaagaugagcuccauauagggagaacugcucagauuggccaugucuauccugcagcaaucagcagcuuugaucgcccacugugggcagagcccugucuuggggagaccagagaaccggaagacccagccccugcccucaaggagcuuuuugucuugccgggggaaccaaggucacagcugcaccaacucccgaagaacccucuuuccgagcugccugucgucaaauccaagcgaguggcauuaagccuugaagaugauggacuacccugaggaugggaucacccccuucgugccucauggaauucagucccaugcacuacacucuggaugguguaugacuggaugaauggguuucuauauaugggucugugugaguguaugugugugugugauuuuuuuuuuaaauuuauguugcggaaagguaaccacaaaguuaugaugaacugcaaacauccaaaggaugugagaguuuuucuauguauaauguuuuauacacuuuuuaacugguugcacuacccaugaggaauucguggaauggcuacugcugacuaacaugaugcacauaaccaaaugggggccaauggcacaguaccuuacucaucauuuaaaaacuauauuuacagaagauguuugguugcugggggggcuuuuuuagguuuuggggcauuuguuuuuuguaaauaagaugauuaugcuuuguggcuauccaucaacauaaguaaaaaaaaaaaaaaaacacuucaacucccucccccauuuagauuauuuauuaacauauuuuaaaaaucagaugaguucuauaaauaauuuagagaagugagaguauuuauuuuuggcauguuuggcccaccacacagacucuguguguguauguguguguuuauauguguaugugugugacagaaaaaucuguagagaagaggcacaucuauggcuacuguucaaauacauaaagauaaauuuauuuucacacaguccacaagggguauaucuuguaguuuucagaaaagccuuuggaaaucuggaucagaaaauagauaccaugguuugugcaauuauguaguaaaaaaggcaaaucuuuucaccucuggcuauuccugagaccccaggaagucaggaaaagccuuucagcucacccauggcugcugugacuccuaccagggcuuucuuggcuuuggcgaaggucaguguacagacauuccaugguaccagagugcucagaaacucaagauaggauaugccucacccucagcuacuccuuguuuuaaaguucagcucuuugaguaacuucuucaauuucuuucaggacacuuggguugaauucaguaaguuuccucugaagcacccugaagggugccauccuuacagagcuaaguggagacguuuccagaucagcccaaguuuacuauagagacuggcccaggcacugaaugucuaggacaugcuguggaugaagauaaagaugguggaauagguuuuaucacaucucuuauuucucuuuuccccuuacucucuaccauuuccuuuauguggggaaacauuuuaagguaauaaauagguuacuuaccaucauauguucauauagaugaaacuaauuuuuggcuuaagucagaacaacuggccaaaauugaagucauauuugaggggggaaauggcauacgcaauauuauauuauauuggauauuuauguucacacaggaauuugguuuacugcuuuguaaauaaaaggaaaaacuccggguauauguauagauguucuucauuauagacaucuucuuugcuuuucuuggccuugggggaggaagggagaagugcucuuuucuacuuguggggucucccauuggaaacauaauccuauagucccagaaggauucaguccccaguggcuuucccauccaaagagaaagaguuugaguuucuuaacucugcuguucugccacuuacucccacuagacaaccagggacaaggugcaacauggaaguguuugacuuaaguaggagcagaggagcugcaucuaaucucaucauaccuggaacuugacacacuuaagcaaaugccuucccaucccuaccugccagaugcccccaacucaaugaaguuggaugucucaccagcuugauacccuuugaauuuucagucagacauucuggaguucuagcauccuguaccuaggaccuuccucugugucacucuuggccuccuaaacucuaagaaaauaacuauauucuggagcuugggcaguguguuuugcauaauccagcaaucuccucaugacaugcauguguugauaguccugaaacauucauugagaggguaaaugcaguugaccuagaaugaccaauaccaaacagaauuuuaagaacagguggccaacuccuauggagcuuacucacauauuacuauucuuuuaagaacggaaaguaaaauuauuuuugacugaagaaaaaugaugacagugaaaaacauggaaauguacucaaaacaagugacuuuuucuguaaccuuccaaagaaacugaauuuuccaaggaauuaaaugauaacaguggcuaaggcauaguuucuaaacuuucaguaagauccuggcauucacagaaaaaaaugaugaauggggucuggacauacagccugagaucucaaaaugacaaugaaauucacaacuuuuucucagagacauucauguuuccugcauaugcuacaacugcaguuugaaagaggcagcaaugggagcaacccuuuacaagaaacaaauugugauauauucauguguuggacggcaguaaauaagaugaaaccugaggagucagauccaccuucccccauucauagaggcuuuucagccucauuuugagguacaguuacauaucuuuugccuuuugcccccgugcauagcuaucuacagccaaucacagaucacagagucacuggacuauagagcuggaaggaagcucagagacaaugccaagggggcagaaaauuuaucagaagccagucccagugcguuuccuccauuuccuucugcaggaagacuauuuugggcugccugaacauuguaucaaaccugcuaccuauacuauggucuaccuuuccuccaguggaauuacaaaggcacuaacugaaaugccuucuagaaacagagaaaacgaaacuguacuuauuuacucuugauacacagauuauuuauaaaacagauugaaguaaccuguuaacuggcaaaaagagaaugagaucggauuuaaauguauggcaguaaguccuauugaucccuccaguuaucucaguaugacugcaguauauucauucacuaaaaccacucacuagauaccaacuacacaccuggcacugcagauguaaaggucagucacacauguucugacuuuacagaguucacaguagcaguggaggaugauauauguggaaacaaaaaaggcauugauucuauucagagcacuguuagggcucaaaggagagaggggucuuuccaccuaagaaaugaggaauagggucaucauagaagugaccuuaagucuuaaaaauuaagaaggggauuccaagcugcuucagacagagacacaucgagcuaaaacacagagguaugaaagagcacagggacuuuaggaauugcacaguucauucuaacaggaacaaaaggcucaaggggggcaagaaaugaggcuguauggaaagagauucaauguaagcacuuuauaaaauagauuaauuucugauucaaugaagcauuucuugaucauuguguacaaggcacuacaugcaucauggaaaauucauuaggaugcauugccagcacuuugcagaacugauauuauucagccucaagcuuuccaguggccaaagggaaaugcugacugcuuuucauauauuugagucaaagauuuuuuauauggucaaugaagacuaauauaagggcagugggauuuucacagaugcaugccauguugucgagagccucuuagauuuucucaacugugagaaagaaaaacgaaaauguugaagacguugagucuggagaggggauacuaaucacuguccaguugggcacuggugggaauggggaaauggcacaggaaugcaagccucuccacccuaccccccgaacuccagccauacacucaucguuucacaaaauauaaaugaguuagcauuaaauguuucagaguaaauaauuccuuuucccgaaaugcaugaagauagaguaacagacuucucacacuguauuuuuaggguauggagaauuuagaagguuaaagaauuacugcuucaauuuuucaguuaaaaaaaaaucaggaagcucuguucauucaggcuaugcaccaugugcacagucaagaauuagcagaaacccucugcauuuacaaacacuuugugcuauaaaaaaguaauuuuuaaaaagccacguguguguguguguauauauauauauauauauauauuuaaagccaagguuuugauacuuuuuuacaaaaacuacaagagaaaacaaauauaccuguccaaaccauauacuuuuaaaagagcauuuuuuuuuccauacaagcuguuguuaauuuggggguaaagugcugauuugcaaacuucaucaaauuguucccaaguggauucuccuuguuugucucccccuaccaaccccaaaguuaccauauuugauguaagaaucaggcauguuagaauguugugucacacuaacugauucugcucuuuuugucuugucauucaaguuccguuagcuucuguacgcggugcccuuugcagucuggugucucuuccagaggcgagggggcugaggauggggugcugcaucucacuagcuauacuggcaucaucuugguaaacugaaaaccaaauguggacauuuguaaaaucagugcacuguuucuagagagagauuaaauucauuuaaaaaaaa

SEQ ID NO: 14 - protein, 793 aa, Homo sapiens
MGLPEPGPLRLLALLLLLLLLLLLQLQHLAAAAADPLLGGQGPAKDCEKDQFQCRNERCIPSVWRCDEDDDCLDHSDEDDCPKKTCADSDFTCDNGHCIHERWKCDGEEECPDGSDESEATCTKQVCPAEKLSCGPTSHKCVPASWRCDGEKDCEGGADEAGCATWLNECLHNNGGCSHICTDLKIGFECTCPAGFQLLDQKTCGDIDECKDPDACSQICVNYKGYFKCECYPGYEMDLLTKNCKAAAGKSPSLIFTNRHEVRRIDLVKRNYSRLIPMLKNVVALDVEVATNRIYWCDLSYRKIYSAYMDKASDPKEQEVLIDEQLHSPEGLAVDWVHKHIYWTDSGNKTISVATVDGGRRRTLFSRNLSEPRAIAVDPLRGFMYWSDWGDQAKIEKSGLNGVDRQTLVSDNIEWPNGITLDLLSQRLYWVDSKLHQLSSIDFSGGNRKTLISSTDFLSHPFGIAVFEDKVFWTDLENEAIFSANRLNGLEISILAENLNNPHDIVIFHELKQPRAPDACELSVQPNGGCEYLCLPAPQISSHSPKYTCACPDTMWLGPDMKRCYRAPQSTSTTTLASTMTRTVPATTRAPGTTVHRSTYQNHSTETPSLTAAVPSSVSVPRAPSISPSTLSPATSNHSQHYANEDSKMGSTVTAAVIGIIVPIVVIALLCMSGYLIWRNWKRKNTKSMNFDNPVYRKTTEEEDEDELHIGRTAQIGHVYPAAISSFDRPLWAEPCLGETREPEDPAPALKELFVLPGEPRSQLHQLPKNPLSELPVVKSKRVALSLEDDGLP

SEQ ID NO: 15 - RNA, 6994 nt, Homo sapiens
gcuggcggcggccgcccagggccggggccgcgcgcccagccugagcccgccccgccgccgagcgucaccgaaccugcuugaaaugcagccgaggagccggggcgggcggcagcggcggcggcggcggcggcgggggcagcggcaaccccggcgccgcggcaaggacucggagggcugagacgcggcggcggcggcgcggggagcgcggggcgcggcggccggagccccgggcccgccaugggccuccccgagccgggcccucuccggcuucuggcgcugcugcugcugcugcugcugcugcugcugcugcagcuccagcaucuugcggcggcagcggcugauccgcugcucggcggccaagggccggccaaggauugcgaaaaggaccaauuccagugccggaacgagcgcugcauccccucuguguggagaugcgacgaggacgaugacugcuuagaccacagcgacgaggacgacugccccaagaagaccugugcagacagugacuucaccugugacaacggccacugcauccacgaacgguggaagugugacggcgaggaggaguguccugauggcuccgaugaguccgaggccacuugcaccaagcagguguguccugcagagaagcugagcuguggacccaccagccacaaguguguaccugccucguggcgcugcgacggggagaaggacugcgaggguggagcggaugaggccggcugugcuaccucacugggcaccugccguggggacgaguuccaguguggggaugggacauguguccuugcaaucaagcacugcaaccaggagcaggacuguccagaugggagugaugaagcuggcugccuacaggggcugaacgagugucugcacaacaauggcggcugcucacacaucugcacugaccucaagauuggcuuugaaugcacgugcccagcaggcuuccagcuccuggaccagaagaccuguggcgacauugaugagugcaaggacccagaugccugcagccagaucugugucaauuacaagggcuauuuuaagugugagugcuacccuggcuacgagauggaccuacugaccaagaacugcaaggcugcugcuggcaagagcccaucccuaaucuucaccaaccggcacgaggugcggaggaucgaccuggugaagcggaacuauucacgccucauccccaugcucaagaaugucguggcacuagauguggaaguugccaccaaucgcaucuacuggugugaccucuccuaccguaagaucuauagcgccuacauggacaaggccagugacccgaaagagcaggagguccucauugacgagcaguugcacucuccagagggccuggcaguggacuggguccacaagcacaucuacuggacugacucgggcaauaagaccaucucaguggccacaguugaugguggccgccgacgcacucucuucagccguaaccucagugaaccccgggccaucgcuguugacccccugcgaggguucauguauuggucugacuggggggaccaggccaagauugagaaaucugggcucaacgguguggaccggcaaacacuggugucagacaauauugaauggcccaacggaaucacccuggaucugcugagccagcgcuuguacuggguagacuccaagcuacaccaacuguccagcauugacuucaguggaggcaacagaaagacgcugaucuccuccacugacuuccugagccacccuuuugggauagcuguguuugaggacaagguguucuggacagaccuggagaacgaggccauuuucagugcaaaucggcucaauggccuggaaaucuccauccuggcugagaaccucaacaacccacaugacauugucaucuuccaugagcugaagcagccaagagcuccagaugccugugagcugaguguccagccuaauggaggcugugaauaccugugccuuccugcuccucagaucuccagccacucucccaaguacacaugugccuguccugacacaauguggcuggguccagacaugaagaggugcuaccgagaugcaaaugaagacaguaagaugggcucaacagucacugccgcuguuaucgggaucaucgugcccauaguggugauagcccuccugugcaugaguggauaccugaucuggagaaacuggaagcggaagaacaccaaaagcaugaauuuugacaacccagucuacaggaaaacaacagaagaagaagacgaagaugagcuccauauagggagaacugcucagauuggccaugucuauccugcacgaguggcauuaagccuugaagaugauggacuacccugaggaugggaucacccccuucgugccucauggaauucagucccaugcacuacacucuggaugguguaugacuggaugaauggguuucuauauaugggucugugugaguguaugugugugugugauuuuuuuuuuaaauuuauguugcggaaagguaaccacaaaguuaugaugaacugcaaacauccaaaggaugugagaguuuuucuauguauaauguuuuauacacuuuuuaacugguugcacuacccaugaggaauucguggaauggcuacugcugacuaacaugaugcacauaaccaaaugggggccaauggcacaguaccuuacucaucauuuaaaaacuauauuuacagaagauguuugguugcugggggggcuuuuuuagguuuuggggcauuuguuuuuuguaaauaagaugauuaugcuuuguggcuauccaucaacauaaguaaaaaaaaaaaaaaaacacuucaacucccucccccauuuagauuauuuauuaacauauuuuaaaaaucagaugaguucuauaaauaauuuagagaagugagaguauuuauuuuuggcauguuuggcccaccacacagacucuguguguguauguguguguuuauauguguaugugugugacagaaaaaucuguagagaagaggcacaucuauggcuacuguucaaauacauaaagauaaauuuauuuucacacaguccacaagggguauaucuuguaguuuucagaaaagccuuuggaaaucuggaucagaaaauagauaccaugguuugugcaauuauguaguaaaaaaggcaaaucuuuucaccucuggcuauuccugagaccccaggaagucaggaaaagccuuucagcucacccauggcugcugugacuccuaccagggcuuucuuggcuuuggcgaaggucaguguacagacauuccaugguaccagagugcucagaaacucaagauaggauaugccucacccucagcuacuccuuguuuuaaaguucagcucuuugaguaacuucuucaauuucuuucaggacacuuggguugaauucaguaaguuuccucugaagcacccugaagggugccauccuuacagagcuaaguggagacguuuccagaucagcccaaguuuacuauagagacuggcccaggcacugaaugucuaggacaugcuguggaugaagauaaagaugguggaauagguuuuaucacaucucuuauuucucuuuuccccuuacucucuaccauuuccuuuauguggggaaacauuuuaagguaauaaauagguuacuuaccaucauauguucauauagaugaaacuaauuuuuggcuuaagucagaacaacuggccaaaauugaagucauauuugaggggggaaauggcauacgcaauauuauauuauauuggauauuuauguucacacaggaauuugguuuacugcuuuguaaauaaaaggaaaaacuccggguauauguauagauguucuucauuauagacaucuucuuugcuuuucuuggccuugggggaggaagggagaagugcucuuuucuacuuguggggucucccauuggaaacauaauccuauagucccagaaggauucaguccccaguggcuuucccauccaaagagaaagaguuugaguuucuuaacucugcuguucugccacuuacucccacuagacaaccagggacaaggugcaacauggaaguguuugacuuaaguaggagcagaggagcugcaucuaaucucaucauaccuggaacuugacacacuuaagcaaaugccuucccaucccuaccugccagaugcccccaacucaaugaaguuggaugucucaccagcuugauacccuuugaauuuucagucagacauucuggaguucuagcauccuguaccuaggaccuuccucugugucacucuuggccuccuaaacucuaagaaaauaacuauauucuggagcuugggcaguguguuuugcauaauccagcaaucuccucaugacaugcauguguugauaguccugaaacauucauugagaggguaaaugcaguugaccuagaaugaccaauaccaaacagaauuuuaagaacagguggccaacuccuauggagcuuacucacauauuacuauucuuuuaagaacggaaaguaaaauuauuuuugacugaagaaaaaugaugacagugaaaaacauggaaauguacucaaaacaagugacuuuuucuguaaccuuccaaagaaacugaauuuuccaaggaauuaaaugauaacaguggcuaaggcauaguuucuaaacuuucaguaagauccuggcauucacagaaaaaaaugaugaauggggucuggacauacagccugagaucucaaaaugacaaugaaauucacaacuuuuucucagagacauucauguuuccugcauaugcuacaacugcaguuugaaagaggcagcaaugggagcaacccuuuacaagaaacaaauugugauauauucauguguuggacggcaguaaauaagaugaaaccugaggagucagauccaccuucccccauucauagaggcuuuucagccucauuuugagguacaguuacauaucuuuugccuuuugcccccgugcauagcuaucuacagccaaucacagaucacagagucacuggacuauagagcuggaaggaagcucagagacaaugccaagggggcagaaaauuuaucagaagccagucccagugcguuuccuccauuuccuucugcaggaagacuauuuugggcugccugaacauuguaucaaaccugcuaccuauacuauggucuaccuuuccuccaguggaauuacaaaggcacuaacugaaaugccuucuagaaacagagaaaacgaaacuguacuuauuuacucuugauacacagauuauuuauaaaacagauugaaguaaccuguuaacuggcaaaaagagaaugagaucggauuuaaauguauggcaguaaguccuauugaucccuccaguuaucucaguaugacugcaguauauucauucacuaaaaccacucacuagauaccaacuacacaccuggcacugcagauguaaaggucagucacacauguucugacuuuacagaguucacaguagcaguggaggaugauauauguggaaacaaaaaaggcauugauucuauucagagcacuguuagggcucaaaggagagaggggucuuuccaccuaagaaaugaggaauagggucaucauagaagugaccuuaagucuuaaaaauuaagaaggggauuccaagcugcuucagacagagacacaucgagcuaaaacacagagguaugaaagagcacagggacuuuaggaauugcacaguucauucuaacaggaacaaaaggcucaaggggggcaagaaaugaggcuguauggaaagagauucaauguaagcacuuuauaaaauagauuaauuucugauucaaugaagcauuucuugaucauuguguacaaggcacuacaugcaucauggaaaauucauuaggaugcauugccagcacuuugcagaacugauauuauucagccucaagcuuuccaguggccaaagggaaaugcugacugcuuuucauauauuugagucaaagauuuuuuauauggucaaugaagacuaauauaagggcagugggauuuucacagaugcaugccauguugucgagagccucuuagauuuucucaacugugagaaagaaaaacgaaaauguugaagacguugagucuggagaggggauacuaaucacuguccaguugggcacuggugggaauggggaaauggcacaggaaugcaagccucuccacccuaccccccgaacuccagccauacacucaucguuucacaaaauauaaaugaguuagcauuaaauguuucagaguaaauaauuccuuuucccgaaaugcaugaagauagaguaacagacuucucacacuguauuuuuaggguauggagaauuuagaagguuaaagaauuacugcuucaauuuuucaguuaaaaaaaaaucaggaagcucuguucauucaggcuaugcaccaugugcacagucaagaauuagcagaaacccucugcauuuacaaacacuuugugcuauaaaaaaguaauuuuuaaaaagccacguguguguguguguauauauauauauauauauauauuuaaagccaagguuuugauacuuuuuuacaaaaacuacaagagaaaacaaauauaccuguccaaaccauauacuuuuaaaagagcauuuuuuuuuccauacaagcuguuguuaauuuggggguaaagugcugauuugcaaacuucaucaaauuguucccaaguggauucuccuuguuugucucccccuaccaaccccaaaguuaccauauuugauguaagaaucaggcauguuagaauguugugucacacuaacugauucugcucuuuuugucuugucauucaaguuccguuagcuucuguacgcggugcccuuugcagucuggugucucuuccagaggcgagggggcugaggauggggugcugcaucucacuagcuauacuggcaucaucuugguaaacugaaaaccaaauguggacauuuguaaaaucagugcacuguuucuagagagagauuaaauucauuuaaaaaaaa

SEQ ID NO: 16 - protein, 700 aa, Homo sapiens
MGLPEPGPLRLLALLLLLLLLLLLQLQHLAAAAADPLLGGQGPAKDCEKDQFQCRNERCIPSVWRCDEDDDCLDHSDEDDCPKKTCADSDFTCDNGHCIHERWKCDGEEECPDGSDESEATCTKQVCPAEKLSCGPTSHKCVPASWRCDGEKDCEGGADEAGCATSLGTCRGDEFQCGDGTCVLAIKHCNQEQDCPDGSDEAGCLQGLNECLHNNGGCSHICTDLKIGFECTCPAGFQLLDQKTCGDIDECKDPDACSQICVNYKGYFKCECYPGYEMDLLTKNCKAAAGKSPSLIFTNRHEVRRIDLVKRNYSRLIPMLKNVVALDVEVATNRIYWCDLSYRKIYSAYMDKASDPKEQEVLIDEQLHSPEGLAVDWVHKHIYWTDSGNKTISVATVDGGRRRTLFSRNLSEPRAIAVDPLRGFMYWSDWGDQAKIEKSGLNGVDRQTLVSDNIEWPNGITLDLLSQRLYWVDSKLHQLSSIDFSGGNRKTLISSTDFLSHPFGIAVFEDKVFWTDLENEAIFSANRLNGLEISILAENLNNPHDIVIFHELKQPRAPDACELSVQPNGGCEYLCLPAPQISSHSPKYTCACPDTMWLGPDMKRCYRDANEDSKMGSTVTAAVIGIIVPIVVIALLCMSGYLIWRNWKRKNTKSMNFDNPVYRKTTEEEDEDELHIGRTAQIGHVYPARVALSLEDDGLP

SEQ ID NO: 17 - RNA, 7606 nt, Homo sapiens
gcuggcggcggccgcccagggccggggccgcgcgcccagccugagcccgccccgccgccgagcgucaccgaaccugcuugaaaugcagccgaggagccggggcgggcggcagcggcggcggcggcggcggcgggggcagcggcaaccccggcgccgcggcaaggacucggagggcugagacgcggcggcggcggcgcggggagcgcggggcgcggcggccggagccccgggcccgccaugggccuccccgagccgggcccucuccggcuucuggcgcugcugcugcugcugcugcugcugcugcugcugcagcuccagcaucuugcggcggcagcggcugauccgcugcucggcggccaagggccggccaaggauugcgaaaaggaccaauuccagugccggaacgagcgcugcauccccucuguguggagaugcgacgaggacgaugacugcuuagaccacagcgacgaggacgacugccccaagaagaccugugcagacagugacuucaccugugacaacggccacugcauccacgaacgguggaagugugacggcgaggaggaguguccugauggcuccgaugaguccgaggccacuugcaccaagcagguguguccugcagagaagcugagcuguggacccaccagccacaaguguguaccugccucguggcgcugcgacggggagaaggacugcgaggguggagcggaugaggccggcugugcuaccuugugcgccccgcacgaguuccagugcggcaaccgcucgugccuggccgccguguucgugugcgacggcgacgacgacuguggugacggcagcgaugagcgcggcugugcagacccggccugcgggccccgcgaguuccgcugcggcggcgauggcggcggcgccugcaucccggagcgcugggucugcgaccgccaguuugacugcgaggaccgcucggacgaggcagccgagcucugcggccguccgggccccggggccacguccgcgcccgccgccugcgccaccgccucccaguucgccugccgcagcggcgagugcgugcaccugggcuggcgcugcgacggcgaccgcgacugcaaagacaaaucggacgaggccgacugcccacugggcaccugccguggggacgaguuccaguguggggaugggacauguguccuugcaaucaagcacugcaaccaggagcaggacuguccagaugggagugaugaagcuggcugccuacaggggcugaacgagugucugcacaacaauggcggcugcucacacaucugcacugaccucaagauuggcuuugaaugcacgugcccagcaggcuuccagcuccuggaccagaagaccuguggcgacauugaugagugcaaggacccagaugccugcagccagaucugugucaauuacaagggcuauuuuaagugugagugcuacccuggcuacgagauggaccuacugaccaagaacugcaaggcugcugcuggcaagagcccaucccuaaucuucaccaaccggcacgaggugcggaggaucgaccuggugaagcggaacuauucacgccucauccccaugcucaagaaugucguggcacuagauguggaaguugccaccaaucgcaucuacuggugugaccucuccuaccguaagaucuauagcgccuacauggacaaggccagugacccgaaagagcaggagguccucauugacgagcaguugcacucuccagagggccuggcaguggacuggguccacaagcacaucuacuggacugacucgggcaauaagaccaucucaguggccacaguugaugguggccgccgacgcacucucuucagccguaaccucagugaaccccgggccaucgcuguugacccccugcgaggguucauguauuggucugacuggggggaccaggccaagauugagaaaucugggcucaacgguguggaccggcaaacacuggugucagacaauauugaauggcccaacggaaucacccuggaucugcugagccagcgcuuguacuggguagacuccaagcuacaccaacuguccagcauugacuucaguggaggcaacagaaagacgcugaucuccuccacugacuuccugagccacccuuuugggauagcuguguuugaggacaagguguucuggacagaccuggagaacgaggccauuuucagugcaaaucggcucaauggccuggaaaucuccauccuggcugagaaccucaacaacccacaugacauugucaucuuccaugagcugaagcagccaagagcuccagaugccugugagcugaguguccagccuaauggaggcugugaauaccugugccuuccugcuccucagaucuccagccacucucccaaguacacaugugccuguccugacacaauguggcuggguccagacaugaagaggugcuaccgagcaccucaaucuaccucaacuacgacguuagcuucuaccaugacgaggacaguaccugccaccacaagagcccccgggaccaccguccacagauccaccuaccagaaccacagcacagagacaccaagccugacagcugcagucccaagcucaguuaguguccccagggcucccagcaucagcccgucuacccuaagcccugcaaccagcaaccacucccagcacuaugcaaaugaagacaguaagaugggcucaacagucacugccgcuguuaucgggaucaucgugcccauaguggugauagcccuccugugcaugaguggauaccugaucuggagaaacuggaagcggaagaacaccaaaagcaugaauuuugacaacccagucuacaggaaaacaacagaagaagaagacgaagaugagcuccauauagggagaacugcucagauuggccaugucuauccugcacgaguggcauuaagccuugaagaugauggacuacccugaggaugggaucacccccuucgugccucauggaauucagucccaugcacuacacucuggaugguguaugacuggaugaauggguuucuauauaugggucugugugaguguaugugugugugugauuuuuuuuuuaaauuuauguugcggaaagguaaccacaaaguuaugaugaacugcaaacauccaaaggaugugagaguuuuucuauguauaauguuuuauacacuuuuuaacugguugcacuacccaugaggaauucguggaauggcuacugcugacuaacaugaugcacauaaccaaaugggggccaauggcacaguaccuuacucaucauuuaaaaacuauauuuacagaagauguuugguugcugggggggcuuuuuuagguuuuggggcauuuguuuuuuguaaauaagaugauuaugcuuuguggcuauccaucaacauaaguaaaaaaaaaaaaaaaacacuucaacucccucccccauuuagauuauuuauuaacauauuuuaaaaaucagaugaguucuauaaauaauuuagagaagugagaguauuuauuuuuggcauguuuggcccaccacacagacucuguguguguauguguguguuuauauguguaugugugugacagaaaaaucuguagagaagaggcacaucuauggcuacuguucaaauacauaaagauaaauuuauuuucacacaguccacaagggguauaucuuguaguuuucagaaaagccuuuggaaaucuggaucagaaaauagauaccaugguuugugcaauuauguaguaaaaaaggcaaaucuuuucaccucuggcuauuccugagaccccaggaagucaggaaaagccuuucagcucacccauggcugcugugacuccuaccagggcuuucuuggcuuuggcgaaggucaguguacagacauuccaugguaccagagugcucagaaacucaagauaggauaugccucacccucagcuacuccuuguuuuaaaguucagcucuuugaguaacuucuucaauuucuuucaggacacuuggguugaauucaguaaguuuccucugaagcacccugaagggugccauccuuacagagcuaaguggagacguuuccagaucagcccaaguuuacuauagagacuggcccaggcacugaaugucuaggacaugcuguggaugaagauaaagaugguggaauagguuuuaucacaucucuuauuucucuuuuccccuuacucucuaccauuuccuuuauguggggaaacauuuuaagguaauaaauagguuacuuaccaucauauguucauauagaugaaacuaauuuuuggcuuaagucagaacaacuggccaaaauugaagucauauuugaggggggaaauggcauacgcaauauuauauuauauuggauauuuauguucacacaggaauuugguuuacugcuuuguaaauaaaaggaaaaacuccggguauauguauagauguucuucauuauagacaucuucuuugcuuuucuuggccuugggggaggaagggagaagugcucuuuucuacuuguggggucucccauuggaaacauaauccuauagucccagaaggauucaguccccaguggcuuucccauccaaagagaaagaguuugaguuucuuaacucugcuguucugccacuuacucccacuagacaaccagggacaaggugcaacauggaaguguuugacuuaaguaggagcagaggagcugcaucuaaucucaucauaccuggaacuugacacacuuaagcaaaugccuucccaucccuaccugccagaugcccccaacucaaugaaguuggaugucucaccagcuugauacccuuugaauuuucagucagacauucuggaguucuagcauccuguaccuaggaccuuccucugugucacucuuggccuccuaaacucuaagaaaauaacuauauucuggagcuugggcaguguguuuugcauaauccagcaaucuccucaugacaugcauguguugauaguccugaaacauucauugagaggguaaaugcaguugaccuagaaugaccaauaccaaacagaauuuuaagaacagguggccaacuccuauggagcuuacucacauauuacuauucuuuuaagaacggaaaguaaaauuauuuuugacugaagaaaaaugaugacagugaaaaacauggaaauguacucaaaacaagugacuuuuucuguaaccuuccaaagaaacugaauuuuccaaggaauuaaaugauaacaguggcuaaggcauaguuucuaaacuuucaguaagauccuggcauucacagaaaaaaaugaugaauggggucuggacauacagccugagaucucaaaaugacaaugaaauucacaacuuuuucucagagacauucauguuuccugcauaugcuacaacugcaguuugaaagaggcagcaaugggagcaacccuuuacaagaaacaaauugugauauauucauguguuggacggcaguaaauaagaugaaaccugaggagucagauccaccuucccccauucauagaggcuuuucagccucauuuugagguacaguuacauaucuuuugccuuuugcccccgugcauagcuaucuacagccaaucacagaucacagagucacuggacuauagagcuggaaggaagcucagagacaaugccaagggggcagaaaauuuaucagaagccagucccagugcguuuccuccauuuccuucugcaggaagacuauuuugggcugccugaacauuguaucaaaccugcuaccuauacuauggucuaccuuuccuccaguggaauuacaaaggcacuaacugaaaugccuucuagaaacagagaaaacgaaacuguacuuauuuacucuugauacacagauuauuuauaaaacagauugaaguaaccuguuaacuggcaaaaagagaaugagaucggauuuaaauguauggcaguaaguccuauugaucccuccaguuaucucaguaugacugcaguauauucauucacuaaaaccacucacuagauaccaacuacacaccuggcacugcagauguaaaggucagucacacauguucugacuuuacagaguucacaguagcaguggaggaugauauauguggaaacaaaaaaggcauugauucuauucagagcacuguuagggcucaaaggagagaggggucuuuccaccuaagaaaugaggaauagggucaucauagaagugaccuuaagucuuaaaaauuaagaaggggauuccaagcugcuucagacagagacacaucgagcuaaaacacagagguaugaaagagcacagggacuuuaggaauugcacaguucauucuaacaggaacaaaaggcucaaggggggcaagaaaugaggcuguauggaaagagauucaauguaagcacuuuauaaaauagauuaauuucugauucaaugaagcauuucuugaucauuguguacaaggcacuacaugcaucauggaaaauucauuaggaugcauugccagcacuuugcagaacugauauuauucagccucaagcuuuccaguggccaaagggaaaugcugacugcuuuucauauauuugagucaaagauuuuuuauauggucaaugaagacuaauauaagggcagugggauuuucacagaugcaugccauguugucgagagccucuuagauuuucucaacugugagaaagaaaaacgaaaauguugaagacguugagucuggagaggggauacuaaucacuguccaguugggcacuggugggaauggggaaauggcacaggaaugcaagccucuccacccuaccccccgaacuccagccauacacucaucguuucacaaaauauaaaugaguuagcauuaaauguuucagaguaaauaauuccuuuucccgaaaugcaugaagauagaguaacagacuucucacacuguauuuuuaggguauggagaauuuagaagguuaaagaauuacugcuucaauuuuucaguuaaaaaaaaaucaggaagcucuguucauucaggcuaugcaccaugugcacagucaagaauuagcagaaacccucugcauuuacaaacacuuugugcuauaaaaaaguaauuuuuaaaaagccacguguguguguguguauauauauauauauauauauauuuaaagccaagguuuugauacuuuuuuacaaaaacuacaagagaaaacaaauauaccuguccaaaccauauacuuuuaaaagagcauuuuuuuuuccauacaagcuguuguuaauuuggggguaaagugcugauuugcaaacuucaucaaauuguucccaaguggauucuccuuguuugucucccccuaccaaccccaaaguuaccauauuugauguaagaaucaggcauguuagaauguugugucacacuaacugauucugcucuuuuugucuugucauucaaguuccguuagcuucuguacgcggugcccuuugcagucuggugucucuuccagaggcgagggggcugaggauggggugcugcaucucacuagcuauacuggcaucaucuugguaaacugaaaaccaaauguggacauuuguaaaaucagugcacuguuucuagagagagauuaaauucauuuaaaaaaaa

SEQ ID NO: 18 - protein, 904 aa, Homo sapiens
MGLPEPGPLRLLALLLLLLLLLLLQLQHLAAAAADPLLGGQGPAKDCEKDQFQCRNERCIPSVWRCDEDDDCLDHSDEDDCPKKTCADSDFTCDNGHCIHERWKCDGEEECPDGSDESEATCTKQVCPAEKLSCGPTSHKCVPASWRCDGEKDCEGGADEAGCATLCAPHEFQCGNRSCLAAVFVCDGDDDCGDGSDERGCADPACGPREFRCGGDGGGACIPERWVCDRQFDCEDRSDEAAELCGRPGPGATSAPAACATASQFACRSGECVHLGWRCDGDRDCKDKSDEADCPLGTCRGDEFQCGDGTCVLAIKHCNQEQDCPDGSDEAGCLQGLNECLHNNGGCSHICTDLKIGFECTCPAGFQLLDQKTCGDIDECKDPDACSQICVNYKGYFKCECYPGYEMDLLTKNCKAAAGKSPSLIFTNRHEVRRIDLVKRNYSRLIPMLKNVVALDVEVATNRIYWCDLSYRKIYSAYMDKASDPKEQEVLIDEQLHSPEGLAVDWVHKHIYWTDSGNKTISVATVDGGRRRTLFSRNLSEPRAIAVDPLRGFMYWSDWGDQAKIEKSGLNGVDRQTLVSDNIEWPNGITLDLLSQRLYWVDSKLHQLSSIDFSGGNRKTLISSTDFLSHPFGIAVFEDKVFWTDLENEAIFSANRLNGLEISILAENLNNPHDIVIFHELKQPRAPDACELSVQPNGGCEYLCLPAPQISSHSPKYTCACPDTMWLGPDMKRCYRAPQSTSTTTLASTMTRTVPATTRAPGTTVHRSTYQNHSTETPSLTAAVPSSVSVPRAPSISPSTLSPATSNHSQHYANEDSKMGSTVTAAVIGIIVPIVVIALLCMSGYLIWRNWKRKNTKSMNFDNPVYRKTTEEEDEDELHIGRTAQIGHVYPARVALSLEDDGLP

SEQ ID NO: 19 - RNA, 2358 nt, Homo sapiens
aaacucacacaacaacucuuccccgcugagaggagacagccagugcgacuccacccuccagcucgacggcagccgccccggccgacagccccgagacgacagcccggcgcgucccgguccccaccuccgaccaccgccagcgcuccaggccccgccgcuccccgcucgccgccaccgcgcccuccgcuccgcccgcagugccaaccaugaccgccgccaguaugggccccguccgcgucgccuucgugguccuccucgcccucugcagccggccggccgucggccagaacugcagcgggccgugccggugcccggacgagccggcgccgcgcugcccggcgggcgugagccucgugcuggacggcugcggcugcugccgcgucugcgccaagcagcugggcgagcugugcaccgagcgcgaccccugcgacccgcacaagggccucuucugugacuucggcuccccggccaaccgcaagaucggcgugugcaccgccaaagauggugcucccugcaucuucggugguacgguguaccgcagcggagaguccuuccagagcagcugcaaguaccagugcacgugccuggacggggcggugggcugcaugccccugugcagcauggacguucgucugcccagcccugacugccccuucccgaggagggucaagcugcccgggaaaugcugcgaggagugggugugugacgagcccaaggaccaaaccgugguugggccugcccucgcggcuuaccgacuggaagacacguuuggcccagacccaacuaugauuagagccaacugccugguccagaccacagaguggagcgccuguuccaagaccugugggaugggcaucuccacccggguuaccaaugacaacgccuccugcaggcuagagaagcagagccgccugugcauggucaggccuugcgaagcugaccuggaagagaacauuaagaagggcaaaaagugcauccguacucccaaaaucuccaagccuaucaaguuugagcuuucuggcugcaccagcaugaagacauaccgagcuaaauucuguggaguauguaccgacggccgaugcugcaccccccacagaaccaccacccugccgguggaguucaagugcccugacggcgaggucaugaagaagaacaugauguucaucaagaccugugccugccauuacaacugucccggagacaaugacaucuuugaaucgcuguacuacaggaagauguacggagacauggcaugaagccagagagugagagacauuaacucauuagacuggaacuugaacugauucacaucucauuuuuccguaaaaaugauuucaguagcacaaguuauuuaaaucuguuuuucuaacugggggaaaagauucccacccaauucaaaacauugugccaugucaaacaaauagucuaucaaccccagacacugguuugaagaauguuaagacuugacaguggaacuacauuaguacacagcaccagaauguauauuaagguguggcuuuaggagcagugggaggguaccagcagaaagguuaguaucaucagauagcaucuuauacgaguaauaugccugcuauuugaaguguaauugagaaggaaaauuuuagcgugcucacugaccugccuguagccccagugacagcuaggaugugcauucuccagccaucaagagacugagucaaguuguuccuuaagucagaacagcagacucagcucugacauucugauucgaaugacacuguucaggaaucggaauccugucgauuagacuggacagcuuguggcaagugaauuugccuguaacaagccagauuuuuuaaaauuuauauuguaaauauuguguguguguguguguguguauauauauauauauguacaguuaucuaaguuaauuuaaaguuguuugugccuuuuuauuuuuguuuuuaaugcuuugauauuucaauguuagccucaauuucugaacaccauagguagaauguaaagcuugucugaucguucaaagcaugaaauggauacuuauauggaaauucugcucagauagaaugacaguccgucaaaacagauuguuugcaaaggggaggcaucaguguccuuggcaggcugauuucuagguaggaaaugugguagccucacuuuuaaugaacaaauggccuuuauuaaaaacugagugacucuauauagcugaucaguuuuuucaccuggaagcauuuguuucuacuuugauaugacuguuuuucggacaguuuauuuguugagagugugaccaaaaguuacauguuugcaccuuucuaguugaaaauaaaguguauauuuuuucuauaaaaaaaaaaaaaaaaa

SEQ ID NO: 20 - protein, 349 aa, Homo sapiens
MTAASMGPVRVAFVVLLALCSRPAVGQNCSGPCRCPDEPAPRCPAGVSLVLDGCGCCRVCAKQLGELCTERDPCDPHKGLFCDFGSPANRKIGVCTAKDGAPCIFGGTVYRSGESFQSSCKYQCTCLDGAVGCMPLCSMDVRLPSPDCPFPRRVKLPGKCCEEWVCDEPKDQTVVGPALAAYRLEDTFGPDPTMIRANCLVQTTEWSACSKTCGMGISTRVTNDNASCRLEKQSRLCMVRPCEADLEENIKKGKKCIRTPKISKPIKFELSGCTSMKTYRAKFCGVCTDGRCCTPHRTTTLPVEFKCPDGEVMKKNMMFIKTCACHYNCPGDNDIFESLYYRKMYGDMA

SEQ ID NO: 21 - RNA, 1939 nt, Homo sapiens
aggaaggagggguggccugaccccucggcagucccuccccucagccuuuccccaaauugcuacuucucuggggcuccagguccugcuugugcucagcuccagcucacuggcuggccaccgagacuucuggacaggaaacugcaccauccucuucucccagcaagggggcuccagagacugcccacccaggaagucugguggccuggggauuuggacagugccuugguaaugaccagggcuccaggaagagauguccuuguggcugggggccccugugccugacauuccuccugacucugcgguggagcuguggaagccaggcgcacaggaugcaagcagccaggcccagggaggcagcagcugcauccucagagaggaagccaggaugccccacucugcuggggguacugcagggguggggcuggaggcugcagagcccacagcccugcucaccagggcagagcccccuucagaacccacagagauccguccacaaaagcggaaaaaggggccagcccccaaaaugcuggggaacgagcuaugcagcguguguggggacaaggccucgggcuuccacuacaauguucugagcugcgagggcugcaagggauucuuccgccgcagcgucaucaagggagcgcacuacaucugccacaguggcggccacugccccauggacaccuacaugcgucgcaagugccaggagugucggcuucgcaaaugccgucaggcuggcaugcgggaggaguguguccugucagaagaacagauccgccugaagaaacugaagcggcaagaggaggaacaggcucaugccacauccuugccccccagggcuuccucacccccccaaauccugccccagcucagcccggaacaacugggcaugaucgagaagcucgucgcugcccagcaacaguguaaccggcgcuccuuuucugaccggcuucgagucacgccuuggcccauggcaccagauccccauagccgggaggcccgucagcagcgcuuugcccacuucacugagcuggccaucgucucugugcaggagauaguugacuuugcuaaacagcuacccggcuuccugcagcucagccgggaggaccagauugcccugcugaagaccucugcgaucgaggugaugcuucuggagacaucucggagguacaacccugggagugagaguaucaccuuccucaaggauuucaguuauaaccgggaagacuuugccaaagcagggcugcaaguggaauucaucaaccccaucuucgaguucuccagggccaugaaugagcugcaacucaaugaugccgaguuugccuugcucauugcuaucagcaucuucucugcagaccggcccaacgugcaggaccagcuccagguagagaggcugcagcacacauauguggaagcccugcaugccuacgucuccauccaccauccccaugaccgacugauguucccacggaugcuaaugaaacuggugagccuccggacccugagcagcguccacucagagcaaguguuugcacugcgucugcaggacaaaaagcucccaccgcugcucucugagaucugggaugugcacgaaugacuguucuguccccauauuuucuguuuucuuggccggauggcugaggccugguggcugccuccuagaaguggaacagacugagaagggcaaacauuccugggagcugggcaaggagauccucccguggcauuaaaagagagucaaaggguugcgaguuuuguggcuacugagcaguggagcccucgcuaacacugugcugugucugaagaucaugcugaccccacaaacggaugggccugggggccacuuugcacaggguucuccagagcccugcccauccugccuccaccacuuccuguuuuucccacagggccccaagaaaaauucuccacugucaaaaaaaaa

SEQ ID NO: 22 - protein, 447 aa, Homo sapiens
MSLWLGAPVPDIPPDSAVELWKPGAQDASSQAQGGSSCILREEARMPHSAGGTAGVGLEAAEPTALLTRAEPPSEPTEIRPQKRKKGPAPKMLGNELCSVCGDKASGFHYNVLSCEGCKGFFRRSVIKGAHYICHSGGHCPMDTYMRRKCQECRLRKCRQAGMREECVLSEEQIRLKKLKRQEEEQAHATSLPPRASSPPQILPQLSPEQLGMIEKLVAAQQQCNRRSFSDRLRVTPWPMAPDPHSREARQQRFAHFTELAIVSVQEIVDFAKQLPGFLQLSREDQIALLKTSAIEVMLLETSRRYNPGSESITFLKDFSYNREDFAKAGLQVEFINPIFEFSRAMNELQLNDAEFALLIAISIFSADRPNVQDQLQVERLQHTYVEALHAYVSIHHPHDRLMFPRMLMKLVSLRTLSSVHSEQVFALRLQDKKLPPLLSEIWDVHE

SEQ ID NO: 23 - RNA, 1759 nt, Homo sapiens
aggaaggagggguggccugaccccucggcagucccuccccucagccuuuccccaaauugcuacuucucuggggcuccagguccugcuugugcucagcuccagcucacuggcuggccaccgagacuucuggacaggaaacugcaccauccucuucucccagcaagggggcuccagagacugcccacccaggaagucugguggccuggggauuuggacagugccuugguaaugaccagggcuccaggaagagauguccuuguggcugggggccccugugccugacauuccuccugacucugcgguggagcuguggaagccaggcgcacaggaugcaagcagccaggcccagggaggcagcagcugcauccucagagaggaagccaggaugccccacucugcuggggguacugcagggguggggcuggaggcugcagagcccacagcccugcucaccagggcagagcccccuucagaacccacagagauccguccacaaaagcggaaaaaggggccagcccccaaaaugcuggggaacgagcuaugcagcguguguggggacaaggccucgggcuuccacuacaauguucugagcugcgagggcugcaagggauucuuccgccgcagcgucaucaagggagcgcacuacaucugccacaguggcggccacugccccauggacaccuacaugcgucgcaagugccaggagugucggcuucgcaaaugccgucaggcuggcaugcgggaggaguguguccugucagaagaacagauccgccugaagaaacugaagcggcaagaggaggaacaggcucaugccacauccuugccccccagggcuuccucacccccccaaauccugccccagcucagcccggaacaacugggcaugaucgagaagcucgucgcugcccagcaacaguguaaccggcgcuccuuuucugaccggcuucgagucacggugaugcuucuggagacaucucggagguacaacccugggagugagaguaucaccuuccucaaggauuucaguuauaaccgggaagacuuugccaaagcagggcugcaaguggaauucaucaaccccaucuucgaguucuccagggccaugaaugagcugcaacucaaugaugccgaguuugccuugcucauugcuaucagcaucuucucugcagaccggcccaacgugcaggaccagcuccagguagagaggcugcagcacacauauguggaagcccugcaugccuacgucuccauccaccauccccaugaccgacugauguucccacggaugcuaaugaaacuggugagccuccggacccugagcagcguccacucagagcaaguguuugcacugcgucugcaggacaaaaagcucccaccgcugcucucugagaucugggaugugcacgaaugacuguucuguccccauauuuucuguuuucuuggccggauggcugaggccugguggcugccuccuagaaguggaacagacugagaagggcaaacauuccugggagcugggcaaggagauccucccguggcauuaaaagagagucaaaggguugcgaguuuuguggcuacugagcaguggagcccucgcuaacacugugcugugucugaagaucaugcugaccccacaaacggaugggccugggggccacuuugcacaggguucuccagagcccugcccauccugccuccaccacuuccuguuuuucccacagggccccaagaaaaauucuccacugucaaaaaaaaa

SEQ ID NO: 24 - protein, 387 aa, Homo sapiens
MSLWLGAPVPDIPPDSAVELWKPGAQDASSQAQGGSSCILREEARMPHSAGGTAGVGLEAAEPTALLTRAEPPSEPTEIRPQKRKKGPAPKMLGNELCSVCGDKASGFHYNVLSCEGCKGFFRRSVIKGAHYICHSGGHCPMDTYMRRKCQECRLRKCRQAGMREECVLSEEQIRLKKLKRQEEEQAHATSLPPRASSPPQILPQLSPEQLGMIEKLVAAQQQCNRRSFSDRLRVTVMLLETSRRYNPGSESITFLKDFSYNREDFAKAGLQVEFINPIFEFSRAMNELQLNDAEFALLIAISIFSADRPNVQDQLQVERLQHTYVEALHAYVSIHHPHDRLMFPRMLMKLVSLRTLSSVHSEQVFALRLQDKKLPPLLSEIWDVHE

SEQ ID NO: 25 - RNA, 1748 nt, Homo sapiens
aucuuacuuagggaccugcuggggugcggggaaaaggcgcagucucggugggauugcgugcaggagggucguggucuggcuguggcggaggagcauaagaagacucugcgguggagcuguggaagccaggcgcacaggaugcaagcagccaggcccagggaggcagcagcugcauccucagagaggaagccaggaugccccacucugcuggggguacugcagggguggggcuggaggcugcagagcccacagcccugcucaccagggcagagcccccuucagaacccacagagauccguccacaaaagcggaaaaaggggccagcccccaaaaugcuggggaacgagcuaugcagcguguguggggacaaggccucgggcuuccacuacaauguucugagcugcgagggcugcaagggauucuuccgccgcagcgucaucaagggagcgcacuacaucugccacaguggcggccacugccccauggacaccuacaugcgucgcaagugccaggagugucggcuucgcaaaugccgucaggcuggcaugcgggaggaguguguccugucagaagaacagauccgccugaagaaacugaagcggcaagaggaggaacaggcucaugccacauccuugccccccagggcuuccucacccccccaaauccugccccagcucagcccggaacaacugggcaugaucgagaagcucgucgcugcccagcaacaguguaaccggcgcuccuuuucugaccggcuucgagucacgccuuggcccauggcaccagauccccauagccgggaggcccgucagcagcgcuuugcccacuucacugagcuggccaucgucucugugcaggagauaguugacuuugcuaaacagcuacccggcuuccugcagcucagccgggaggaccagauugcccugcugaagaccucugcgaucgaggugaugcuucuggagacaucucggagguacaacccugggagugagaguaucaccuuccucaaggauuucaguuauaaccgggaagacuuugccaaagcagggcugcaaguggaauucaucaaccccaucuucgaguucuccagggccaugaaugagcugcaacucaaugaugccgaguuugccuugcucauugcuaucagcaucuucucugcagaccggcccaacgugcaggaccagcuccagguagagaggcugcagcacacauauguggaagcccugcaugccuacgucuccauccaccauccccaugaccgacugauguucccacggaugcuaaugaaacuggugagccuccggacccugagcagcguccacucagagcaaguguuugcacugcgucugcaggacaaaaagcucccaccgcugcucucugagaucugggaugugcacgaaugacuguucuguccccauauuuucuguuuucuuggccggauggcugaggccugguggcugccuccuagaaguggaacagacugagaagggcaaacauuccugggagcugggcaaggagauccucccguggcauuaaaagagagucaaaggguugcgaguuuuguggcuacugagcaguggagcccucgcuaacacugugcugugucugaagaucaugcugaccccacaaacggaugggccugggggccacuuugcacaggguucuccagagcccugcccauccugccuccaccacuuccuguuuuucccacagggccccaagaaaaauucuccacugucaaaaaaaaa

SEQ ID NO: 26 - protein, 402 aa, Homo sapiens
MPHSAGGTAGVGLEAAEPTALLTRAEPPSEPTEIRPQKRKKGPAPKMLGNELCSVCGDKASGFHYNVLSCEGCKGFFRRSVIKGAHYICHSGGHCPMDTYMRRKCQECRLRKCRQAGMREECVLSEEQIRLKKLKRQEEEQAHATSLPPRASSPPQILPQLSPEQLGMIEKLVAAQQQCNRRSFSDRLRVTPWPMAPDPHSREARQQRFAHFTELAIVSVQEIVDFAKQLPGFLQLSREDQIALLKTSAIEVMLLETSRRYNPGSESITFLKDFSYNREDFAKAGLQVEFINPIFEFSRAMNELQLNDAEFALLIAISIFSADRPNVQDQLQVERLQHTYVEALHAYVSIHHPHDRLMFPRMLMKLVSLRTLSSVHSEQVFALRLQDKKLPPLLSEIWDVHE

SEQ ID NO: 27 - RNA, 1928 nt, Homo sapiens
gauucuaacuuagcuaagcaaugcuacuggagaccauaggcaaagccaagguacagcuucagggaagucuuuggugagcccaucucucauuaccaagguaacgaagcgcagacuccgggcccgggugggcggcaucaccaccagguucacgccgagaaggagcuggaggagagccgcccggcuccagccggaccgcuugcccgccaucaccguuguaaucuaugcagcaaacaagcuggaacccgcuggguggcaccugcaagcagccgcccggacgcacccacucugcgguggagcuguggaagccaggcgcacaggaugcaagcagccaggcccagggaggcagcagcugcauccucagagaggaagccaggaugccccacucugcuggggguacugcagggguggggcuggaggcugcagagcccacagcccugcucaccagggcagagcccccuucagaacccacagagauccguccacaaaagcggaaaaaggggccagcccccaaaaugcuggggaacgagcuaugcagcguguguggggacaaggccucgggcuuccacuacaauguucugagcugcgagggcugcaagggauucuuccgccgcagcgucaucaagggagcgcacuacaucugccacaguggcggccacugccccauggacaccuacaugcgucgcaagugccaggagugucggcuucgcaaaugccgucaggcuggcaugcgggaggaguguguccugucagaagaacagauccgccugaagaaacugaagcggcaagaggaggaacaggcucaugccacauccuugccccccagggcuuccucacccccccaaauccugccccagcucagcccggaacaacugggcaugaucgagaagcucgucgcugcccagcaacaguguaaccggcgcuccuuuucugaccggcuucgagucacgccuuggcccauggcaccagauccccauagccgggaggcccgucagcagcgcuuugcccacuucacugagcuggccaucgucucugugcaggagauaguugacuuugcuaaacagcuacccggcuuccugcagcucagccgggaggaccagauugcccugcugaagaccucugcgaucgaggugaugcuucuggagacaucucggagguacaacccugggagugagaguaucaccuuccucaaggauuucaguuauaaccgggaagacuuugccaaagcagggcugcaaguggaauucaucaaccccaucuucgaguucuccagggccaugaaugagcugcaacucaaugaugccgaguuugccuugcucauugcuaucagcaucuucucugcagaccggcccaacgugcaggaccagcuccagguagagaggcugcagcacacauauguggaagcccugcaugccuacgucuccauccaccauccccaugaccgacugauguucccacggaugcuaaugaaacuggugagccuccggacccugagcagcguccacucagagcaaguguuugcacugcgucugcaggacaaaaagcucccaccgcugcucucugagaucugggaugugcacgaaugacuguucuguccccauauuuucuguuuucuuggccggauggcugaggccugguggcugccuccuagaaguggaacagacugagaagggcaaacauuccugggagcugggcaaggagauccucccguggcauuaaaagagagucaaaggguugcgaguuuuguggcuacugagcaguggagcccucgcuaacacugugcugugucugaagaucaugcugaccccacaaacggaugggccugggggccacuuugcacaggguucuccagagcccugcccauccugccuccaccacuuccuguuuuucccacagggccccaagaaaaauucuccacugucaaaaaaaaa

SEQ ID NO: 28 - protein, 453 aa, Homo sapiens
MQQTSWNPLGGTCKQPPGRTHSAVELWKPGAQDASSQAQGGSSCILREEARMPHSAGGTAGVGLEAAEPTALLTRAEPPSEPTEIRPQKRKKGPAPKMLGNELCSVCGDKASGFHYNVLSCEGCKGFFRRSVIKGAHYICHSGGHCPMDTYMRRKCQECRLRKCRQAGMREECVLSEEQIRLKKLKRQEEEQAHATSLPPRASSPPQILPQLSPEQLGMIEKLVAAQQQCNRRSFSDRLRVTPWPMAPDPHSREARQQRFAHFTELAIVSVQEIVDFAKQLPGFLQLSREDQIALLKTSAIEVMLLETSRRYNPGSESITFLKDFSYNREDFAKAGLQVEFINPIFEFSRAMNELQLNDAEFALLIAISIFSADRPNVQDQLQVERLQHTYVEALHAYVSIHHPHDRLMFPRMLMKLVSLRTLSSVHSEQVFALRLQDKKLPPLLSEIWDVHE

SEQ ID NO: 29 - RNA, 2093 nt, Homo sapiens
ucgucaaguuucacgcuccgccccucuuccggacgugacgcaagggcgggguugccggaagaaguggcgaaguuacuuuugaggguauuugaguagcggcggugugucaggggcuaaagaggaggacgaagaaaagcagagcaagggaacccagggcaacaggaguaguucacuccgcgagaggccguccacgagacccccgcgcgcagccaugagccccgccccccgcuguugcuuggagaggggcgggaccuggagagaggcugcuccgugaccccaccauguccucuccuaccacgaguucccuggauaccccccugccuggaaauggccccccucagccuggcgccccuucuucuucacccacuguaaaggaggaggguccggagccguggcccggggguccggacccugaugucccaggcacugaugaggccagcucagccugcagcacagacugggucaucccagaucccgaagaggaaccagagcgcaagcgaaagaagggcccagccccgaagaugcugggccacgagcuuugccgugucuguggggacaaggccuccggcuuccacuacaacgugcucagcugcgaaggcugcaagggcuucuuccggcgcagugugguccgugguggggccaggcgcuaugccugccgggguggcggaaccugccagauggacgcuuucaugcggcgcaagugccagcagugccggcugcgcaagugcaaggaggcagggaugagggagcagugcguccuuucugaagaacagauccggaagaagaagauucggaaacaacagcagcaggagucacagucacagucgcagucaccuguggggccgcagggcagcagcagcucagccucugggccuggggcuuccccugguggaucugaggcaggcagccagggcuccggggaaggcgaggguguccagcuaacagcggcucaagaacuaaugauccagcaguugguggcggcccaacugcagugcaacaaacgcuccuucuccgaccagcccaaagucacgcccuggccccugggcgcagacccccagucccgagaugcccgccagcaacgcuuugcccacuucacggagcuggccaucaucucaguccaggagaucguggacuucgcuaagcaagugccugguuuccugcagcugggccgggaggaccagaucgcccuccugaaggcauccacuaucgagaucaugcugcuagagacagccaggcgcuacaaccacgagacagaguguaucaccuucuugaaggacuucaccuacagcaaggacgacuuccaccgugcaggccugcagguggaguucaucaaccccaucuucgaguucucgcgggccaugcggcggcugggccuggacgacgcugaguacgcccugcucaucgccaucaacaucuucucggccgaccggcccaacgugcaggagccgggccgcguggaggcguugcagcagcccuacguggaggcgcugcuguccuacacgcgcaucaagaggccgcaggaccagcugcgcuucccgcgcaugcucaugaagcuggugagccugcgcacgcugagcucugugcacucggagcaggucuucgccuugcggcuccaggacaagaagcugccgccucugcugucggagaucugggacguccacgagugaggggcuggccacccagccccacagccuugccugaccacccuccagcagauagacgccggcaccccuuccucuuccuaggguggaaggggcccugggccgagccuguagaccuaucggcucucaucccuugggauaagccccaguccagguccaggaggcucccucccugcccagcgagucuuccagaaggggugaaaggguugcaggucccgaccacugacccuucccggcugcccucccuccccagcuuacaccucaagcccagcacgcagugcaccuugaacagagggaggggaggacccauggcucuccccccuagcccgggagaccagggccuuccucuuccucugcuuuuauuuaauaaaaacuaaaaacagaaacaggaaaauaaaauaugaauacaauccagcccggagcuggagugca

SEQ ID NO: 30 - protein, 461 aa, Homo sapiens
MSSPTTSSLDTPLPGNGPPQPGAPSSSPTVKEEGPEPWPGGPDPDVPGTDEASSACSTDWVIPDPEEEPERKRKKGPAPKMLGHELCRVCGDKASGFHYNVLSCEGCKGFFRRSVVRGGARRYACRGGGTCQMDAFMRRKCQQCRLRKCKEAGMREQCVLSEEQIRKKKIRKQQQQESQSQSQSPVGPQGSSSSASGPGASPGGSEAGSQGSGEGEGVQLTAAQELMIQQLVAAQLQCNKRSFSDQPKVTPWPLGADPQSRDARQQRFAHFTELAIISVQEIVDFAKQVPGFLQLGREDQIALLKASTIEIMLLETARRYNHETECITFLKDFTYSKDDFHRAGLQVEFINPIFEFSRAMRRLGLDDAEYALLIAINIFSADRPNVQEPGRVEALQQPYVEALLSYTRIKRPQDQLRFPRMLMKLVSLRTLSSVHSEQVFALRLQDKKLPPLLSEIWDVHE

SEQ ID NO: 31 - RNA, 1802 nt, Homo sapiens
ucgucaaguuucacgcuccgccccucuuccggacgugacgcaagggcgggguugccggaagaaguggcgaaguuacuuuugaggguauuugaguagcggcggugugucaggggcuaaagaggaggacgaagaaaagcagagcaagggaacccagggcaacaggaguaguucacuccgcgagaggccguccacgagacccccgcgcgcagccaugagccccgccccccgcuguugcuuggagaggggcgggaccuggagagaggcugcuccgugaccccaccauguccucuccuaccacgaguucccuggauaccccccugccuggaaauggccccccucagccuggcgccccuucuucuucacccacuguaaaggaggaggguccggagccguggcccggggguccggacccugaugucccaggcacugaugaggccagcucagccugcagcacagacuggggcguccuuucugaagaacagauccggaagaagaagauucggaaacaacagcagcaggagucacagucacagucgcagucaccuguggggccgcagggcagcagcagcucagccucugggccuggggcuuccccugguggaucugaggcaggcagccagggcuccggggaaggcgaggguguccagcuaacagcggcucaagaacuaaugauccagcaguugguggcggcccaacugcagugcaacaaacgcuccuucuccgaccagcccaaagucacgcccuggccccugggcgcagacccccagucccgagaugcccgccagcaacgcuuugcccacuucacggagcuggccaucaucucaguccaggagaucguggacuucgcuaagcaagugccugguuuccugcagcugggccgggaggaccagaucgcccuccugaaggcauccacuaucgagaucaugcugcuagagacagccaggcgcuacaaccacgagacagaguguaucaccuucuugaaggacuucaccuacagcaaggacgacuuccaccgugcaggccugcagguggaguucaucaaccccaucuucgaguucucgcgggccaugcggcggcugggccuggacgacgcugaguacgcccugcucaucgccaucaacaucuucucggccgaccggcccaacgugcaggagccgggccgcguggaggcguugcagcagcccuacguggaggcgcugcuguccuacacgcgcaucaagaggccgcaggaccagcugcgcuucccgcgcaugcucaugaagcuggugagccugcgcacgcugagcucugugcacucggagcaggucuucgccuugcggcuccaggacaagaagcugccgccucugcugucggagaucugggacguccacgagugaggggcuggccacccagccccacagccuugccugaccacccuccagcagauagacgccggcaccccuuccucuuccuaggguggaaggggcccugggccgagccuguagaccuaucggcucucaucccuugggauaagccccaguccagguccaggaggcucccucccugcccagcgagucuuccagaaggggugaaaggguugcaggucccgaccacugacccuucccggcugcccucccuccccagcuuacaccucaagcccagcacgcagugcaccuugaacagagggaggggaggacccauggcucuccccccuagcccgggagaccagggccuuccucuuccucugcuuuuauuuaauaaaaacuaaaaacagaaacaggaaaauaaaauaugaauacaauccagcccggagcuggagugca

SEQ ID NO: 32 - protein, 364 aa, Homo sapiens
MSSPTTSSLDTPLPGNGPPQPGAPSSSPTVKEEGPEPWPGGPDPDVPGTDEASSACSTDWGVLSEEQIRKKKIRKQQQQESQSQSQSPVGPQGSSSSASGPGASPGGSEAGSQGSGEGEGVQLTAAQELMIQQLVAAQLQCNKRSFSDQPKVTPWPLGADPQSRDARQQRFAHFTELAIISVQEIVDFAKQVPGFLQLGREDQIALLKASTIEIMLLETARRYNHETECITFLKDFTYSKDDFHRAGLQVEFINPIFEFSRAMRRLGLDDAEYALLIAINIFSADRPNVQEPGRVEALQQPYVEALLSYTRIKRPQDQLRFPRMLMKLVSLRTLSSVHSEQVFALRLQDKKLPPLLSEIWDVHE

SEQ ID NO: 33 - RNA, 71 nt, Homo sapiens
gccaacccaguguucagacuaccuguucaggaggcucucaauguguacaguagucugcacauugguuaggc

SEQ ID NO: 34 - RNA, 110 nt, Homo sapiens
aggaagcuucuggagauccugcuccgucgccccaguguucagacuaccuguucaggacaaugccguuguacaguagucugcacauugguuagacugggcaagggagagca

SEQ ID NO: 35 - RNA, 80 nt, Homo sapiens
cgggaaugccgcggcggggacggcgauugguccguauguguggugccaccggccgccggcuccgccccggcccccgcccc

SEQ ID NO: 36 - RNA, 110 nt, Homo sapiens
uuggauguuggccuaguucuguguggaagacuagugauuuuguuguuuuuagauaacuaaaucgacaacaaaucacagucugccauauggcacaggccaugccucuacag

SEQ ID NO: 37 - RNA, 110 nt, Homo sapiens
cuggauacagaguggaccggcuggccccaucuggaagacuagugauuuuguuguugucuuacugcgcucaacaacaaaucccagucuaccuaauggugccagccaucgca

SEQ ID NO: 38 - RNA, 110 nt, Homo sapiens
agauuagaguggcuguggucuagugcuguguggaagacuagugauuuuguuguucugauguacuacgacaacaagucacagccggccucauagcgcagacucccuucgac

SEQ ID NO: 39 - DNA, 71 bp, Homo sapiens
gatccgacagtagcctgcacattagtcacttcctgtcagtaaccaatgtgcagactactgttttttgaatt

SEQ ID NO: 40 - DNA, 73 bp, Homo sapiens
gatccgcccagtgctcagactacccgtgccttcctgtcaggaacaggtagtctgaacactgggtttttgaatt

SEQ ID NO: 41 - DNA, 69 bp, Homo sapiens
gatccgcggcgggaacggcgatcggcccttcctgtcaggaccaatcgccgtccccgccgtttttgaatt

SEQ ID NO: 42 - DNA, 73 bp, Homo sapiens
gatccgtggaagattagtgagtttattatcttcctgtcagacaacaaaatcactagtcttccatttttgaatt

SEQ ID NO: 43 - protein, 14 aa, Mus musculus
TQQIRLQAEIFQAR

SEQ ID NO: 44 - protein, 14 aa, Homo sapiens
AQQIRLQAEAFQAR

SEQ ID NO: 45 - protein, 14 aa, Artificial
  Synthetic
TAQIRLQAEIFQAR

SEQ ID NO: 46 - protein, 14 aa, Artificial
  Synthetic
TQAIRLQAEIFQAR

SEQ ID NO: 47 - protein, 14 aa, Artificial
  Synthetic
TQQARLQAEIFQAR

SEQ ID NO: 48 - protein, 14 aa, Artificial
  Synthetic
TQQIALQAEIFQAR

SEQ ID NO: 49 - protein, 15 aa, Artificial
  Synthetic
QTQQIRLQAEIFQAR

SEQ ID NO: 50 - protein, 13 aa, Artificial
  Synthetic
QQIRLQAEIFQAR

SEQ ID NO: 51 - DNA, 57 bp, Artificial
  Synthetic shAPOE
ccgggaaggagttgaaggcctacaactcgagttgtaggccttcaactccttcttttt

SEQ ID NO: 52 - DNA, 57 bp, Artificial
  Synthetic shAPOE
ccgggcagacactgtctgagcaggtctcgagacctgctcagacagtgtctgcttttt

SEQ ID NO: 53 - DNA, 57 bp, Artificial
  Synthetic shDNAJA
ccgggcgagaagtttaaactcatatctcgagatatgagtttaaacttctcgcttttt

SEQ ID NO: 54 - DNA, 57 bp, Artificial
  Synthetic shDNAJA4
ccggcctcgacagaaagtgaggattctcgagaatcctcactttctgtcgaggttttt

SEQ ID NO: 55 - DNA, 30 bp, Artificial
  Synthetic ApoE Forward Primer
tcatgaggatccatgaaggttctgtgggct

SEQ ID NO: 56 - DNA, 29 bp, Artificial
  Synthetic ApoE Reverse Primer
tagcagaattctcagtgattgtcgctggg

SEQ ID NO: 57 - DNA, 31 bp, Artificial
  Synthetic DNAJA4 Forward Primer
atccctggatccatgtgggaaagcctgaccc

SEQ ID NO: 58 - DNA, 31 bp, Artificial
  Synthetic DNAJA4 Reverse Primer
taccatgtcgactcatgccgtctggcactgc

SEQ ID NO: 59 - RNA, 19 nt, Artificial
  Synthetic LRP1 target sequence
cgaggacgaugacugcuua

SEQ ID NO: 60 - RNA, 19 nt, Artificial
  Synthetic LRP1 target sequence
gcuaugaguuuaagaaguu

SEQ ID NO: 61 - RNA, 19 nt, Artificial
  Synthetic LRP8 target sequence
cgaggacgaugacugcuua

SEQ ID NO: 62 - RNA, 19 nt, Artificial
  Synthetic LRP8 target sequence
gaacuauucacgccucauc

SEQ ID NO: 63 - DNA, 20 bp, Artificial
  Synthetic ApoE Forward Primer
tgggtcgcttttgggattac

SEQ ID NO: 64 - DNA, 21 bp, Artificial
  Synthetic ApoE Reverse Primer
ttcaactccttcatggtctcg

SEQ ID NO: 65 - DNA, 20 bp, Artificial
  Synthetic DNAJA4 Forward Primer
ccagcttctcttcacccatg

SEQ ID NO: 66 - DNA, 20 bp, Artificial
  Synthetic DNAJA4 Reverse Primer
gccaatttcttcgtgactcc

SEQ ID NO: 67 - DNA, 19 bp, Artificial
  Synthetic GAPDH Forward Primer
agccacatcgctcagacac

SEQ ID NO: 68 - DNA, 19 bp, Artificial
  Synthetic GAPDH Synthetic Primer
gcccaatacgaccaaatcc

SEQ ID NO: 69 - DNA, 21 bp, Artificial
  Synthetic LRP1 Forward Primer
tttaacagcaccgagtaccag

SEQ ID NO: 70 - DNA, 19 bp, Artificial
  Synthetic LRP1 Reverse Primer
caggcagatgtcagagcag

SEQ ID NO: 71 - DNA, 20 bp, Artificial
  Synthetic LRP8 Forward Primer
gctaccctggctacgagatg

SEQ ID NO: 72 - DNA, 20 bp, Artificial
  Synthetic LRP8 Reverse Primer
gattagggatgggctcttgc

SEQ ID NO: 73 - DNA, 8 bp, Artificial
  Synthetic miRNA seed sequence
caguaguc

SEQ ID NO: 74 - DNA, 8 bp, Artificial
  Synthetic miRNA seed sequence
ccaguguu

SEQ ID NO: 75 - DNA, 8 bp, Artificial
  Synthetic miRNA seed sequence
ggcgggga

SEQ ID NO: 76 - DNA, 31 bp, Artificial
  Synthetic Primer
agtacctcgaggggatccttgagtcctactc

SEQ ID NO: 77 - DNA, 34 bp, Artificial
  Synthetic Primer
taattgcggccgctcagacagtgtctgcacccag

SEQ ID NO: 78 - DNA, 31 bp, Artificial
  Synthetic Primer
taatatctcgagatgtgggaaagcctgaccc

SEQ ID NO: 79 - DNA, 32 bp, Artificial
  Synthetic Primer
caattgcggccgctcatgccgtctggcactgc

SEQ ID NO: 80 - DNA, 30 bp, Artificial
  Synthetic Primer
ttagcctcgagacgccgaagcctgcagcca

SEQ ID NO: 81 - DNA, 35 bp, Artificial
  Synthetic Primer
ttactgcggccgctgcgtgaaacttggtgaatctt

SEQ ID NO: 82 - DNA, 30 bp, Artificial
  Synthetic Primer
taatatctcgagcgtggtgcggggcagcgt

SEQ ID NO: 83 - DNA, 35 bp, Artificial
  Synthetic Primer
caattgcggccgcttatctctcataccagctcaat

SEQ ID NO: 84 - DNA, 43 bp, Artificial
  Synthetic Primer
gccagcgctgggaactggcaactggtcgcttttgggattacct

SEQ ID NO: 85 - DNA, 43 bp, Artificial
  Synthetic Primer
cagcgggagaccctgtccccataccagccgtcctcctggggtg

SEQ ID NO: 86 - DNA, 43 bp, Artificial
  Synthetic Primer
tccccgccccagccgtcctcacagggtggaccctagtttaata

SEQ ID NO: 87 - DNA, 43 bp, Artificial
  Synthetic Primer
gggatcggtggagaagtgcctattgtgcaaggggcgggggatg

SEQ ID NO: 88 - DNA, 43 bp, Artificial
  Synthetic Primer
gtagggggcggggaacgtgttatccgtgaagaggtggctaggg

SEQ ID NO: 89 - DNA, 43 bp, Artificial
  Synthetic Primer
cagggccaacttagttcctaacattctgtgcccttcagtggat

SEQ ID NO: 90 - DNA, 43 bp, Artificial
  Synthetic Primer
acagtttgtatggactactatcttaaattatagcttgtttgga

SEQ ID NO: 91 - DNA, 43 bp, Artificial
  Synthetic Primer
taattattgctaaagaactatgttttagttggtaatggtgtaa

SEQ ID NO: 92 - DNA, 45 bp, Artificial
  Synthetic Primer
cagctgcacggaccaggttccataaaaacattgccagctagtgag

SEQ ID NO: 93 - DNA, 22 bp, Artificial
  Synthetic primer
tgagtatttttgtggcaactgc

SEQ ID NO: 94 - DNA, 18 bp, Artificial
  Synthetic primer
ctctgctgggaaagcggc

SEQ ID NO: 95 - DNA, 20 bp, Artificial
  Synthetic primer
caagcactctgcgaactgag

SEQ ID NO: 96 - DNA, 21 bp, Artificial
  Synthetic primer
aagtttttgaaggcaagatgc

SEQ ID NO: 97 - DNA, 23 bp, Artificial
  Synthetic primer
gcggtctggcagtaaaaactatc

SEQ ID NO: 98 - DNA, 23 bp, Artificial
  Synthetic primer
gtgaaacagcattgctgtcactt

SEQ ID NO: 99 - DNA, 24 bp, Artificial
  Synthetic primer
ctaggccacagaattgaaagatct

SEQ ID NO: 100 - DNA, 25 bp, Artificial
  Synthetic primer
gtaggtggaaattctagcatcatcc

SEQ ID NO: 101 - DNA, 20 bp, Artificial
  Synthetic primer
gcctagccgagggagagccg

SEQ ID NO: 102 - DNA, 22 bp, Artificial
  Synthetic primer
tgtgacttgggagctctgcagc

SEQ ID NO: 103 - DNA, 18 bp, Artificial
  Synthetic primer
gccgccccgactgcatct

SEQ ID NO: 104 - DNA, 20 bp, Artificial
  Synthetic primer
tcagtggagggaaggaaatg

SEQ ID NO: 105 - DNA, 20 bp, Artificial
  Synthetic primer
ttcctgccctggacacttac

SEQ ID NO: 106 - DNA, 22 bp, Artificial
  Synthetic primer
ttgtgcccagtcatagccgaat

SEQ ID NO: 107 - DNA, 19 bp, Artificial
  Synthetic primer
ccttttctccctgacaccg

SEQ ID NO: 108 - DNA, 19 bp, Artificial
  Synthetic primer
gcatccatctggcaggttc

SEQ ID NO: 109 - DNA, 20 bp, Artificial
  Synthetic primer
aggtgagatgacaggagatc

SEQ ID NO: 110 - DNA, 57 bp, Artificial
  Synthetic
ccggccgactgatgttcccacggatctcgagatccgtgggaacatcagtcggttttt

SEQ ID NO: 111 - DNA, 57 bp, Artificial
  Synthetic
ccgggcaactcaatgatgccgagttctcgagaactcggcatcattgagttgcttttt

SEQ ID NO: 112 - DNA, 57 bp, Artificial
  Synthetic
ccggagagtgtatcaccttcttgaactcgagttcaagaaggtgatacactctttttt

SEQ ID NO: 113 - DNA, 57 bp, Artificial
  Synthetic
ccgggaaggcatccactatcgagatctcgagatctcgatagtggatgccttcttttt

SEQ ID NO: 114 - DNA, 57 bp, Artificial; identical to SEQ ID NO: 52
  Synthetic

SEQ ID NO: 115 - DNA, 57 bp, Artificial
  Synthetic
ccgggcaactcaatgatgctgagttctcgagaactcagcatcattgagttgcttttt

SEQ ID NO: 116 - DNA, 58 bp, Artificial
  Synthetic
ccggtgagatcatgttgctagaaacctcgaggtttctagcaacatgatctcatttttg

SEQ ID NO: 117 - DNA, 57 bp, Artificial
  Synthetic
ccgggaggacactatgacggaagtactcgagtacttccgtcatagtgtcctcttttt

SEQ ID NO: 118 - DNA, 20 bp, Artificial
  Synthetic primer
tgggtcgcttttgggattac

SEQ ID NO: 119 - DNA, 21 bp, Artificial
  Synthetic primer
ttcaactccttcatggtctcg

SEQ ID NO: 120 - DNA, 19 bp, Artificial
  Synthetic primer
agccacatcgctcagacac

SEQ ID NO: 121 - DNA, 19 bp, Artificial
  Synthetic primer
gcccaatacgaccaaatcc

SEQ ID NO: 122 - DNA, 22 bp, Artificial
  Synthetic primer
gttataaccgggaagactttgc

SEQ ID NO: 123 - DNA, 21 bp, Artificial
  Synthetic primer
aaactcggcatcattgagttg

SEQ ID NO: 124 - DNA, 22 bp, Artificial
  Synthetic primer
tttgagggtatttgagtagcgg

SEQ ID NO: 125 - DNA, 19 bp, Artificial
  Synthetic primer
ctctcgcggagtgaactac

SEQ ID NO: 126 - DNA, 20 bp, Artificial
  Synthetic primer
gaccctggaggctaaggact

SEQ ID NO: 127 - DNA, 20 bp, Artificial
  Synthetic primer
agagccttcatcttcgcaat

SEQ ID NO: 128 - DNA, 20 bp, Artificial
  Synthetic primer
gcacagtcaaggccgagaat

SEQ ID NO: 129 - DNA, 20 bp, Artificial
  Synthetic primer
gccttctccatggtggtgaa

SEQ ID NO: 130 - DNA, 19 bp, Artificial
  Synthetic primer
gcgctcagctcttgtcact

SEQ ID NO: 131 - DNA, 20 bp, Artificial
  Synthetic primer
ctccagccacaaggacatct

SEQ ID NO: 132 - DNA, 20 bp, Artificial
  Synthetic primer
gctctgcctacatcgtggtc

SEQ ID NO: 133 - DNA, 18 bp, Artificial
  Synthetic primer
ctcatggcccagcatctt

SEQ ID NO: 134 - DNA, 19 bp, Artificial
  Synthetic primer
atggagcagggaagaccac

SEQ ID NO: 135 - DNA, 19 bp, Artificial
  Synthetic primer
gtaggccgtgccagaagtt

SEQ ID NO: 136 - DNA, 34 bp, Artificial
  Synthetic primer
tcatagctagcgcagagccaggattcacgccctg

SEQ ID NO: 137 - DNA, 35 bp, Artificial
  Synthetic primer
tggtcctcgaggaaccttcatcttcctgcctgtga

SEQ ID NO: 138 - DNA, 30 bp, Artificial
  Synthetic primer
tagttacgcgtagtagcccccatctttgcc

SEQ ID NO: 139 - DNA, 29 bp, Artificial
  Synthetic primer
aatcagctagcccctcagctgcaaagctc

SEQ ID NO: 140 - DNA, 29 bp, Artificial
  Synthetic primer
tagttacgcgtagtagccccctctttgcc

SEQ ID NO: 141 - DNA, 31 bp, Artificial
  Synthetic primer
aatcagctagcccttcagctgcaaagctctg